European Patent Application EP 4 424 830 A1, published September 4, 2024. Title: Immunoglobulin binding protein. Applicant: 東ソー株式会社. The sequence listing filed with the application follows.

SEQUENCE LISTING (438 sequences)

SEQ ID NO: 1 - protein, 70 aa, Finegoldia magna
ETPEEPKEEVTIKVNLIFADGKIQTAEFKGTFEEATAKAYAYANLLAKENGEYTADLEDGGNTINIKFAG

SEQ ID NO: 2 - DNA, 210 bp, Finegoldia magna
  source 1..210: mol_type = genomic DNA
gaaactcccgaagaaccaaaagaagaagttacgattaaggttaacttaatcttcgccgacggtaagattcagacagctgaatttaagggaacattcgaagaagcgaccgcgaaagcatacgcgtacgccaacctgctggcgaaagaaaacggtgagtataccgccgatttagaagatggcggcaatacgatcaatatcaagtttgcgggt

SEQ ID NO: 3 - DNA, 20 bp, synthetic construct
  misc_feature 1..20: note = PCR forward primer
  source 1..20: mol_type = other DNA
taatacgactcactataggg

SEQ ID NO: 4 - DNA, 19 bp, synthetic construct
  misc_feature 1..19: note = PCR reverse primer
  source 1..19: mol_type = other DNA
tatgctagttattgctcag

SEQ ID NO: 5 - protein, 70 aa, synthetic construct
  REGION 1..70: note = FpL_C3 N62Y
ETPEEPKEEVTIKVNLIFADGKIQTAEFKGTFEEATAKAYAYANLLAKENGEYTADLEDGGYTINIKFAG

SEQ ID NO: 6 - protein, 70 aa, synthetic construct
  REGION 1..70: note = FpL_C3 I17F N50S
ETPEEPKEEVTIKVNLFFADGKIQTAEFKGTFEEATAKAYAYANLLAKESGEYTADLEDGGNTINIKFAG

SEQ ID NO: 7 - protein, 70 aa, synthetic construct
  REGION 1..70: note = FpL_C3 K22R K29R N44S
ETPEEPKEEVTIKVNLIFADGRIQTAEFRGTFEEATAKAYAYASLLAKENGEYTADLEDGGNTINIKFAG

SEQ ID NO: 8 - protein, 70 aa, synthetic construct
  REGION 1..70: note = FpL_C3 E8G E52V N62Y
ETPEEPKGEVTIKVNLIFADGKIQTAEFKGTFEEATAKAYAYANLLAKENGVYTADLEDGGYTINIKFAG

SEQ ID NO: 9 - protein, 70 aa, synthetic construct
  REGION 1..70: note = FpL_C3 E49V
ETPEEPKEEVTIKVNLIFADGKIQTAEFKGTFEEATAKAYAYANLLAKVNGEYTADLEDGGNTINIKFAG

SEQ ID NO: 10 - protein, 70 aa, synthetic construct
  REGION 1..70: note = FpL_C3 K22R
ETPEEPKEEVTIKVNLIFADGRIQTAEFKGTFEEATAKAYAYANLLAKENGEYTADLEDGGNTINIKFAG

SEQ ID NO: 11 - protein, 70 aa, synthetic construct
  REGION 1..70: note = FpL_C3 N50Y E52G (FpL_C3 2a)
ETPEEPKEEVTIKVNLIFADGKIQTAEFKGTFEEATAKAYAYANLLAKEYGGYTADLEDGGNTINIKFAG

SEQ ID NO: 12 - protein, 70 aa, synthetic construct
  REGION 1..70: note = FpL_C3 E27G A41T N50K N65Y
ETPEEPKEEVTIKVNLIFADGKIQTAGFKGTFEEATAKAYTYANLLAKEKGEYTADLEDGGNTIYIKFAG

SEQ ID NO: 13 - protein, 70 aa, synthetic construct
  REGION 1..70: note = FpL_C3 N50S
ETPEEPKEEVTIKVNLIFADGKIQTAEFKGTFEEATAKAYAYANLLAKESGEYTADLEDGGNTINIKFAG

SEQ ID NO: 14 - protein, 70 aa, synthetic construct
  REGION 1..70: note = FpL_C3 E5V
ETPEVPKEEVTIKVNLIFADGKIQTAEFKGTFEEATAKAYAYANLLAKENGEYTADLEDGGNTINIKFAG

SEQ ID NO: 15 - protein, 70 aa, synthetic construct
  REGION 1..70: note = FpL_C3 P3S N50D T54I
ETSEEPKEEVTIKVNLIFADGKIQTAEFKGTFEEATAKAYAYANLLAKEDGEYIADLEDGGNTINIKFAG

SEQ ID NO: 16 - protein, 70 aa, synthetic construct
  REGION 1..70: note = FpL_C3 E52G
ETPEEPKEEVTIKVNLIFADGKIQTAEFKGTFEEATAKAYAYANLLAKENGGYTADLEDGGNTINIKFAG

SEQ ID NO: 17 - protein, 70 aa, synthetic construct
  REGION 1..70: note = FpL_C3 K38R
ETPEEPKEEVTIKVNLIFADGKIQTAEFKGTFEEATARAYAYANLLAKENGEYTADLEDGGNTINIKFAG

SEQ ID NO: 18 - protein, 70 aa, Finegoldia magna
ETPEEPKEEVTIKVNLIFADGKTQTAEFKGTFEEATAEAYRYADLLAKVNGEYTADLEDGGYTINIKFAG

SEQ ID NO: 19 - DNA, 210 bp, Finegoldia magna
  source 1..210: mol_type = genomic DNA
gaaactcccgaagaaccaaaagaagaagttacgattaaggttaacttaatcttcgccgacggtaagacacagacagctgaatttaagggaacattcgaagaagcgaccgcggaagcataccgttacgccgatctgctggcgaaagtgaacggtgagtataccgccgatttagaagatggcggctacacgatcaatatcaagtttgcgggt

SEQ ID NO: 20 - protein, 70 aa, synthetic construct
  REGION 1..70: note = FpL_C4 E1G
GTPEEPKEEVTIKVNLIFADGKTQTAEFKGTFEEATAEAYRYADLLAKVNGEYTADLEDGGYTINIKFAG

SEQ ID NO: 21 - protein, 70 aa, synthetic construct
  REGION 1..70: note = FpL_C4 N50D
ETPEEPKEEVTIKVNLIFADGKTQTAEFKGTFEEATAEAYRYADLLAKVDGEYTADLEDGGYTINIKFAG

SEQ ID NO: 22 - protein, 70 aa, synthetic construct
  REGION 1..70: note = FpL_C4 K22R
ETPEEPKEEVTIKVNLIFADGRTQTAEFKGTFEEATAEAYRYADLLAKVNGEYTADLEDGGYTINIKFAG

SEQ ID NO: 23 - protein, 70 aa, synthetic construct
  REGION 1..70: note = FpL_C3 3a
ETPEEPKEEVTIKVNLIFADGKIQTAEFKGTFEEATAKAYAYANLLAKEYGGYTADLEDGGYTINIKFAG

SEQ ID NO: 24 - DNA, 210 bp, synthetic construct
  misc_feature 1..210: note = FpL_C3 2a DNA
  source 1..210: mol_type = other DNA
gaaactcccgaagaaccaaaagaagaagttacgattaaggttaacttaatcttcgccgacggtaagattcagacagctgaatttaagggaacattcgaagaagcgaccgcgaaagcatacgcgtacgccaacctgctggcgaaagaatacggtgggtataccgccgatttagaagatggcggcaatacgatcaatatcaagtttgcgggt

SEQ ID NO: 25 - DNA, 27 bp, synthetic construct
  misc_feature 1..27: note = PCR forward primer
  source 1..27: mol_type = other DNA
ggcggctatacgatcaatatcaagttt

SEQ ID NO: 26 - DNA, 27 bp, synthetic construct
  misc_feature 1..27: note = PCR reverse primer
  source 1..27: mol_type = other DNA
gatcgtatagccgccatcttctaaatc

SEQ ID NO: 27 - protein, 70 aa, synthetic construct
  REGION 1..70: note = FpL_C3 3b
ETPEEPKEEVTIKVNLIFADGKIQTAEFKGTFEEATAKAYAYANLLAKVYGGYTADLEDGGNTINIKFAG

SEQ ID NO: 28 - DNA, 27 bp, synthetic construct
  misc_feature 1..27: note = PCR forward primer
  source 1..27: mol_type = other DNA
gcgaaagtatacggtgggtataccgcc

SEQ ID NO: 29 - DNA, 27 bp, synthetic construct
  misc_feature 1..27: note = PCR reverse primer
  source 1..27: mol_type = other DNA
accgtatactttcgccagcaggttggc

SEQ ID NO: 30 - protein, 70 aa, synthetic construct
  REGION 1..70: note = FpL_C3 3c
ETPEEPKEEVTIKVNLIFADGKIQTAEFKGTFEEATAKAYAYASLLAKEYGGYTADLEDGGNTINIKFAG

SEQ ID NO: 31 - DNA, 27 bp, synthetic construct
  misc_feature 1..27: note = PCR forward primer
  source 1..27: mol_type = other DNA
tacgccagcctgctggcgaaagaatac

SEQ ID NO: 32 - DNA, 27 bp, synthetic construct
  misc_feature 1..27: note = PCR reverse primer
  source 1..27: mol_type = other DNA
cagcaggctggcgtacgcgtatgcttt

SEQ ID NO: 33 - protein, 70 aa, synthetic construct
  REGION 1..70: note = FpL_C3 3d
ETPEEPKEEVTIKVNLIFADGKIQTAEFKGTFEEATAKAYAYADLLAKEYGGYTADLEDGGNTINIKFAG

SEQ ID NO: 34 - DNA, 27 bp, synthetic construct
  misc_feature 1..27: note = PCR forward primer
  source 1..27: mol_type = other DNA
tacgccgatctgctggcgaaagaatac

SEQ ID NO: 35 - DNA, 27 bp, synthetic construct
  misc_feature 1..27: note = PCR reverse primer
  source 1..27: mol_type = other DNA
cagcagatcggcgtacgcgtatgcttt

SEQ ID NO: 36 - protein, 70 aa, synthetic construct
  REGION 1..70: note = FpL_C3 3e
ETPEEPKEEVTIKVNLIFADGKIQTAEFKGTFEEATAKAYAYANLLAKVYGEYTADLEDGGYTINIKFAG

SEQ ID NO: 37 - DNA, 210 bp, synthetic construct
  misc_feature 1..210: note = FpL_C3 3e DNA
  source 1..210: mol_type = other DNA
gaaaccccggaagaaccaaaggaggaagtcaccatcaaggttaatttgattttcgccgacggtaaaatccagacggcagaattcaaaggaactttcgaagaagcgacagctaaagcgtacgcatacgcaaacctgttagcaaaagtttacggagaatatacggccgatctggaggatggcggctataccattaacatcaagtttgccggg

SEQ ID NO: 38 - protein, 70 aa, synthetic construct
  REGION 1..70: note = FpL_C3 4a
ETPEEPKEEVTIKVNLIFADGKIQTAEFKGTFEEATAKAYAYASLLAKVYGEYTADLEDGGYTINIKFAG

SEQ ID NO: 39 - DNA, 210 bp, synthetic construct
  misc_feature 1..210: note = FpL_C3 4a DNA
  source 1..210: mol_type = other DNA
gaaaccccggaagaaccaaaggaggaagtcaccatcaaggttaatttgattttcgccgacggtaaaatccagacggcagaattcaaaggaactttcgaagaagcgacagctaaagcgtacgcatacgcaagcctgttagcaaaagtttacggagaatatacggccgatctggaggatggcggctataccattaacatcaagtttgccggg

SEQ ID NO: 40 - protein, 70 aa, synthetic construct
  REGION 1..70: note = FpL_C3 4b
ETPEEPKEEVTIKVNLIFADGKIQTAEFKGTFEEATAKAYAYADLLAKVYGEYTADLEDGGYTINIKFAG

SEQ ID NO: 41 - DNA, 210 bp, synthetic construct
  misc_feature 1..210: note = FpL_C3 4b DNA
  source 1..210: mol_type = other DNA
gaaaccccggaagaaccaaaggaggaagtcaccatcaaggttaatttgattttcgccgacggtaaaatccagacggcagaattcaaaggaactttcgaagaagcgacagctaaagcgtacgcatacgcagatctgttagcaaaagtttacggagaatatacggccgatctggaggatggcggctataccattaacatcaagtttgccggg

SEQ ID NO: 42 - protein, 70 aa, synthetic construct
  REGION 1..70: note = FpL_C3 4c
ETPEEPKEEVTIKVNLIFADGKIQTAEFKGTFEEATAKAYAYANLLAKVYGGYTADLEDGGYTINIKFAG

SEQ ID NO: 43 - DNA, 210 bp, synthetic construct
  misc_feature 1..210: note = FpL_C3 4c DNA
  source 1..210: mol_type = other DNA
gaaaccccggaagaaccaaaggaggaagtcaccatcaaggttaatttgattttcgccgacggtaaaatccagacggcagaattcaaaggaactttcgaagaagcgacagctaaagcgtacgcatacgcaaacctgttagcaaaagtttacggaggctatacggccgatctggaggatggcggctataccattaacatcaagtttgccggg

SEQ ID NO: 44 - protein, 70 aa, synthetic construct
  REGION 1..70: note = FpL_C3 4d
ETPEEPKEEVTIKVNLIFADGKIQTAEFKGTFEEATAKAYAYASLLAKEYGGYTADLEDGGYTINIKFAG

SEQ ID NO: 45 - DNA, 210 bp, synthetic construct
  misc_feature 1..210: note = FpL_C3 4d DNA
  source 1..210: mol_type = other DNA
gaaaccccggaagaaccaaaggaggaagtcaccatcaaggttaatttgattttcgccgacggtaaaatccagacggcagaattcaaaggaactttcgaagaagcgacagctaaagcgtacgcatacgcaagcctgttagcaaaagaatacggaggctatacggccgatctggaggatggcggctataccattaacatcaagtttgccggg

SEQ ID NO: 46 - protein, 70 aa, synthetic construct; identical to SEQ ID NO: 40
  REGION 1..70: note = FpL_C3 4e

SEQ ID NO: 47 - DNA, 210 bp, synthetic construct
  misc_feature 1..210: note = FpL_C3 4e DNA
  source 1..210: mol_type = other DNA
gaaaccccggaagaaccaaaggaggaagtcaccatcaaggttaatttgattttcgccgacggtaaaatccagacggcagaattcaaaggaactttcgaagaagcgacagctaaagcgtacgcatacgcagatctgttagcaaaagaatacggaggctatacggccgatctggaggatggcggctataccattaacatcaagtttgccggg

SEQ ID NO: 48 - protein, 70 aa, synthetic construct
  REGION 1..70: note = FpL_C3 5a
ETPEEPKEEVTIKVNLIFADGKIQTAEFKGTFEEATAKAYAYASLLAKVYGGYTADLEDGGYTINIKFAG

SEQ ID NO: 49 - DNA, 210 bp, synthetic construct
  misc_feature 1..210: note = FpL_C3 5a DNA
  source 1..210: mol_type = other DNA
gaaaccccggaagaaccaaaggaggaagtcaccatcaaggttaatttgattttcgccgacggtaaaatccagacggcagaattcaaaggaactttcgaagaagcgacagctaaagcgtacgcatacgcaagcctgttagcaaaagtgtacggaggctatacggccgatctggaggatggcggctataccattaacatcaagtttgccggg

SEQ ID NO: 50 - protein, 70 aa, synthetic construct
  REGION 1..70: note = FpL_C3 5b
ETPEEPKEEVTIKVNLIFADGKIQTAEFKGTFEEATAKAYAYADLLAKVYGGYTADLEDGGYTINIKFAG

SEQ ID NO: 51 - DNA, 210 bp, synthetic construct
  misc_feature 1..210: note = FpL_C3 5b DNA
  source 1..210: mol_type = other DNA
gaaaccccggaagaaccaaaggaggaagtcaccatcaaggttaatttgattttcgccgacggtaaaatccagacggcagaattcaaaggaactttcgaagaagcgacagctaaagcgtacgcatacgcagatctgttagcaaaagtgtacggaggctatacggccgatctggaggatggcggctataccattaacatcaagtttgccggg

SEQ ID NO: 52 - DNA, 80 bp, synthetic construct
  misc_feature 1..80: note = Oligonucleotide
  source 1..80: mol_type = other DNA
ctcgctgcccagccggcgatggccatggaaactcccgaagaaccaaaagaagaagttacgattaaggttaacttaatctt

SEQ ID NO: 53 - DNA, 80 bp, synthetic construct
  misc_feature 1..80: note = Oligonucleotide
  source 1..80: mol_type = other DNA
aagattaagttaaccttaatcgtaacttcttcttttggttcttcgggagtttccatggccatcgccggctgggcagcgag

SEQ ID NO: 54 - DNA, 75 bp, synthetic construct
  misc_feature 1..75: note = Oligonucleotide
  source 1..75: mol_type = other DNA
tacgattaaggttaacttaatcttcgccgacggtaagattcagacagctgaatttaagggaacattcgaagaagc

SEQ ID NO: 55 - DNA, 75 bp, synthetic construct
  misc_feature 1..75: note = Oligonucleotide
  source 1..75: mol_type = other DNA
gcttcttcgaatgttcccttaaattcagctgtctgaatcttaccgtcggcgaagattaagttaaccttaatcgta

SEQ ID NO: 56 - DNA, 77 bp, synthetic construct
  misc_feature 1..77: note = Oligonucleotide
  source 1..77: mol_type = other DNA
aatttaagggaacattcgaagaagcgaccgcgaaagcatacgcgtacgccrrtctgctggcgaaagwawrtggtgda

SEQ ID NO: 57 - DNA, 77 bp, synthetic construct
  misc_feature 1..77: note = Oligonucleotide
  source 1..77: mol_type = other DNA
thcaccaywtwctttcgccagcagayyggcgtacgcgtatgctttcgcggtcgcttcttcgaatgttcccttaaatt

SEQ ID NO: 58 - DNA, 76 bp, synthetic construct
  misc_feature 1..76: note = Oligonucleotide
  source 1..76: mol_type = other DNA
rrtctgctggcgaaagwawrtggtgdatataccgccgatttagaagatggcggcwatacgatcaatatcaagtttg

SEQ ID NO: 59 - DNA, 76 bp, synthetic construct
  misc_feature 1..76: note = Oligonucleotide
  source 1..76: mol_type = other DNA
caaacttgatattgatcgtatwgccgccatcttctaaatcggcggtatathcaccaywtwctttcgccagcagayy

SEQ ID NO: 60 - DNA, 80 bp, synthetic construct
  misc_feature 1..80: note = Oligonucleotide
  source 1..80: mol_type = other DNA
atggcggcwatacgatcaatatcaagtttgcgggtcatcaccaccatcaccactaagcttgcggccgcactcgagcacca

SEQ ID NO: 61 - DNA, 80 bp, synthetic construct
  misc_feature 1..80: note = Oligonucleotide
  source 1..80: mol_type = other DNA
tggtgctcgagtgcggccgcaagcttagtggtgatggtggtgatgacccgcaaacttgatattgatcgtatwgccgccat

SEQ ID NO: 62 - protein, 70 aa, synthetic construct
  REGION 1..70: note = FpL_C3 4f
ETPEEPKEEVTIKVNLIFADGKIQTAEFKGTFEEATAKAYAYADLLAKEYGVYTADLEDGGYTINIKFAG

SEQ ID NO: 63 - protein, 70 aa, synthetic construct
  REGION 1..70: note = FpL_C3 5c
ETPEEPKEEVTIKVNLIFADGKIQTAEFKGTFEEATAKAYAYAGLLAKVYGVYTADLEDGGYTINIKFAG

SEQ ID NO: 64 - protein, 70 aa, synthetic construct
  REGION 1..70: note = FpL_C3 5d
ETPEEPKEEVTIKVNLIFADGKIQTAEFKGTFEEATAKAYAYAGLLAKVSGVYTADLEDGGYTINIKFAG

SEQ ID NO: 65 - DNA, 27 bp, synthetic construct
  misc_feature 1..27: note = G21X forward primer 1
  misc_feature 7: note = n is a, c, g, or t
  misc_feature 8: note = d is a, g, or t
  source 1..27: mol_type = other DNA
gccgacndtaagattcagacagctgaa

SEQ ID NO: 66 - DNA, 27 bp, synthetic construct
  misc_feature 1..27: note = G21X forward primer 2
  source 1..27: mol_type = other DNA
gccgacvhgaagattcagacagctgaa

SEQ ID NO: 67 - DNA, 27 bp, synthetic construct
  misc_feature 1..27: note = G21X forward primer 3
  source 1..27: mol_type = other DNA
gccgactggaagattcagacagctgaa

SEQ ID NO: 68 - DNA, 27 bp, synthetic construct
  misc_feature 1..27: note = G21X reverse primer 1
  misc_feature 8: note = h is a, c, or t
  misc_feature 9: note = n is a, c, g, or t
  source 1..27: mol_type = other DNA
aatcttahngtcggcgaagattaagtt

SEQ ID NO: 69 - DNA, 27 bp, synthetic construct
  misc_feature 1..27: note = G21X reverse primer 2
  source 1..27: mol_type = other DNA
aatcttcdbgtcggcgaagattaagtt

SEQ ID NO: 70 - DNA, 27 bp, synthetic construct
  misc_feature 1..27: note = G21X reverse primer 3
  source 1..27: mol_type = other DNA
aatcttccagtcggcgaagattaagtt

SEQ ID NO: 71 - DNA, 27 bp, synthetic construct
  misc_feature 1..27: note = K22X forward primer 1
  misc_feature 7: note = n is a, c, g, or t
  misc_feature 8: note = d is a, g, or t
  source 1..27: mol_type = other DNA
gacggtndtattcagacagctgaattt

SEQ ID NO: 72 - DNA, 27 bp, synthetic construct
  misc_feature 1..27: note = K22X forward primer 2
  source 1..27: mol_type = other DNA
gacggtvhgattcagacagctgaattt

SEQ ID NO: 73 - DNA, 27 bp, synthetic construct
  misc_feature 1..27: note = K22X forward primer 3
  source 1..27: mol_type = other DNA
gacggttggattcagacagctgaattt

SEQ ID NO: 74 - DNA, 27 bp, synthetic construct
  misc_feature 1..27: note = K22X reverse primer 1
  misc_feature 8: note = h is a, c, or t
  misc_feature 9: note = n is a, c, g, or t
  source 1..27: mol_type = other DNA
ctgaatahnaccgtcggcgaagattaa

SEQ ID NO: 75 - DNA, 27 bp, synthetic construct
  misc_feature 1..27: note = K22X reverse primer 2
  source 1..27: mol_type = other DNA
ctgaatcdbaccgtcggcgaagattaa

SEQ ID NO: 76 - DNA, 27 bp, synthetic construct
  misc_feature 1..27: note = K22X reverse primer 3
  source 1..27: mol_type = other DNA
ctgaatccaaccgtcggcgaagattaa

SEQ ID NO: 77 - DNA, 27 bp, synthetic construct
  misc_feature 1..27: note = T31X forward primer 1
  misc_feature 7: note = n is a, c, g, or t
  misc_feature 8: note = d is a, g, or t
  source 1..27: mol_type = other DNA
aagggandtttcgaagaagcgaccgcg

SEQ ID NO: 78 - DNA, 27 bp, synthetic construct
  misc_feature 1..27: note = T31X forward primer 2
  source 1..27: mol_type = other DNA
aagggavhgttcgaagaagcgaccgcg

SEQ ID NO: 79 - DNA, 27 bp, synthetic construct
  misc_feature 1..27: note = T31X forward primer 3
  source 1..27: mol_type = other DNA
aagggatggttcgaagaagcgaccgcg

SEQ ID NO: 80 - DNA, 27 bp, synthetic construct
  misc_feature 1..27: note = T31X reverse primer 1
  misc_feature 8: note = h is a, c, or t
  misc_feature 9: note = n is a, c, g, or t
  source 1..27: mol_type = other DNA
ttcgaaahntcccttaaattcagctgt

SEQ ID NO: 81 - DNA, 27 bp, synthetic construct
  misc_feature 1..27: note = T31X reverse primer 2
  source 1..27: mol_type = other DNA
ttcgaacdbtcccttaaattcagctgt

SEQ ID NO: 82 - DNA, 27 bp, synthetic construct
  misc_feature 1..27: note = T31X reverse primer 3
  source 1..27: mol_type = other DNA
ttcgaaccatcccttaaattcagctgt

SEQ ID NO: 83 - DNA, 27 bp, synthetic construct
  misc_feature 1..27: note = E49X forward primer 1
  misc_feature 7: note = n is a, c, g, or t
  misc_feature 8: note = d is a, g, or t
  source 1..27: mol_type = other DNA
gcgaaandtaacggtgagtataccgcc

SEQ ID NO: 84 - DNA, 27 bp, synthetic construct
  misc_feature 1..27: note = E49X forward primer 2
  source 1..27: mol_type = other DNA
gcgaaavhgaacggtgagtataccgcc

SEQ ID NO: 85 - DNA, 27 bp, synthetic construct
  misc_feature 1..27: note = E49X forward primer 3
  source 1..27: mol_type = other DNA
gcgaaatggaacggtgagtataccgcc

SEQ ID NO: 86 - DNA, 27 bp, synthetic construct
  misc_feature 1..27: note = E49X reverse primer 1
  misc_feature 8: note = h is a, c, or t
  misc_feature 9: note = n is a, c, g, or t
  source 1..27: mol_type = other DNA
accgttahntttcgccagcaggttggc

SEQ ID NO: 87 - DNA, 27 bp, synthetic construct
  misc_feature 1..27: note = E49X reverse primer 2
  source 1..27: mol_type = other DNA
accgttcdbtttcgccagcaggttggc

SEQ ID NO: 88 - DNA, 27 bp, synthetic construct
  misc_feature 1..27: note = E49X reverse primer 3
  source 1..27: mol_type = other DNA
accgttccatttcgccagcaggttggc

SEQ ID NO: 89 - DNA, 27 bp, synthetic construct
  misc_feature 1..27: note = G51X forward primer 1
  misc_feature 7: note = n is a, c, g, or t
  misc_feature 8: note = d is a, g, or t
  source 1..27: mol_type = other DNA
gaaaacndtgagtataccgccgattta

SEQ ID NO: 90 - DNA, 27 bp, synthetic construct
  misc_feature 1..27: note = G51X forward primer 2
  source 1..27: mol_type = other DNA
gaaaacvhggagtataccgccgattta

SEQ ID NO: 91 - DNA, 27 bp, synthetic construct
  misc_feature 1..27: note = G51X forward primer 3
  source 1..27: mol_type = other DNA
gaaaactgggagtataccgccgattta

SEQ ID NO: 92 - DNA, 27 bp, synthetic construct
  misc_feature 1..27: note = G51X reverse primer 1
  misc_feature 8: note = h is a, c, or t
  misc_feature 9: note = n is a, c, g, or t
  source 1..27: mol_type = other DNA
atactcahngttttctttcgccagcag

SEQ ID NO: 93 - DNA, 27 bp, synthetic construct
  misc_feature 1..27: note = G51X reverse primer 2
  source 1..27: mol_type = other DNA
atactccdbgttttctttcgccagcag

SEQ ID NO: 94 - DNA, 27 bp, synthetic construct
  misc_feature 1..27: note = G51X reverse primer 3
  source 1..27: mol_type = other DNA
atactcccagttttctttcgccagcag

SEQ ID NO: 95 - DNA, 27 bp, synthetic construct
  misc_feature 1..27: note = N62X forward primer 1
  misc_feature 7: note = n is a, c, g, or t
  misc_feature 8: note = d is a, g, or t
  source 1..27: mol_type = other DNA
ggcggcndtacgatcaatatcaagttt

SEQ ID NO: 96 - DNA, 27 bp, synthetic construct
  misc_feature 1..27: note = N62X forward primer 2
  source 1..27: mol_type = other DNA
ggcggcvhgacgatcaatatcaagttt

SEQ ID NO: 97 - DNA, 27 bp, synthetic construct
  misc_feature 1..27: note = N62X forward primer 3
  source 1..27: mol_type = other DNA
ggcggctggacgatcaatatcaagttt

SEQ ID NO: 98 - DNA, 27 bp, synthetic construct
  misc_feature 1..27: note = N62X reverse primer 1
  misc_feature 8: note = h is a, c, or t
  misc_feature 9: note = n is a, c, g, or t
  source 1..27: mol_type = other DNA
gatcgtahngccgccatcttctaaatc

SEQ ID NO: 99 - DNA, 27 bp, synthetic construct
  misc_feature 1..27: note = N62X reverse primer 2
  source 1..27: mol_type = other DNA
gatcgtcdbgccgccatcttctaaatc

SEQ ID NO: 100 - DNA, 27 bp, synthetic construct
  misc_feature 1..27: note = N62X reverse primer 3
  source 1..27: mol_type = other DNA
gatcgtccagccgccatcttctaaatc

SEQ ID NO: 101 - protein, 70 aa, synthetic construct
  REGION 1..70: note = FpL_C3 G21R
ETPEEPKEEVTIKVNLIFADRKIQTAEFKGTFEEATAKAYAYANLLAKENGEYTADLEDGGNTINIKFAG

SEQ ID NO: 102 - protein, 70 aa, synthetic construct
  REGION 1..70: note = FpL_C3 K22T
ETPEEPKEEVTIKVNLIFADGTIQTAEFKGTFEEATAKAYAYANLLAKENGEYTADLEDGGNTINIKFAG

SEQ ID NO: 103 - protein, 70 aa, synthetic construct
  REGION 1..70: note = FpL_C3 T31L
ETPEEPKEEVTIKVNLIFADGKIQTAEFKGLFEEATAKAYAYANLLAKENGEYTADLEDGGNTINIKFAG

SEQ ID NO: 104 - protein, 70 aa, synthetic construct
  REGION 1..70: note = FpL_C3 E49T
ETPEEPKEEVTIKVNLIFADGKIQTAEFKGTFEEATAKAYAYANLLAKTNGEYTADLEDGGNTINIKFAG

SEQ ID NO: 105 - protein, 70 aa, synthetic construct
  REGION 1..70: note = FpL_C3 E49I
ETPEEPKEEVTIKVNLIFADGKIQTAEFKGTFEEATAKAYAYANLLAKINGEYTADLEDGGNTINIKFAG

SEQ ID NO: 106 - protein, 70 aa, synthetic construct
  REGION 1..70: note = FpL_C3 G51V
ETPEEPKEEVTIKVNLIFADGKIQTAEFKGTFEEATAKAYAYANLLAKENVEYTADLEDGGNTINIKFAG

SEQ ID NO: 107 - protein, 70 aa, synthetic construct
  REGION 1..70: note = FpL_C3 N62H
ETPEEPKEEVTIKVNLIFADGKIQTAEFKGTFEEATAKAYAYANLLAKENGEYTADLEDGGHTINIKFAG

SEQ ID NO: 108 - protein, 70 aa, synthetic construct
  REGION 1..70: note = FpL_C3 N62R
ETPEEPKEEVTIKVNLIFADGKIQTAEFKGTFEEATAKAYAYANLLAKENGEYTADLEDGGRTINIKFAG

SEQ ID NO: 109 - protein, 70 aa, synthetic construct
  REGION 1..70: note = FpL_C3 N62L
ETPEEPKEEVTIKVNLIFADGKIQTAEFKGTFEEATAKAYAYANLLAKENGEYTADLEDGGLTINIKFAG

SEQ ID NO: 110 - protein, 70 aa, synthetic construct
  REGION 1..70: note = FpL_C3 N62M
ETPEEPKEEVTIKVNLIFADGKIQTAEFKGTFEEATAKAYAYANLLAKENGEYTADLEDGGMTINIKFAG

SEQ ID NO: 111 - protein, 70 aa, synthetic construct
  REGION 1..70: note = FpL_C3 N62W
ETPEEPKEEVTIKVNLIFADGKIQTAEFKGTFEEATAKAYAYANLLAKENGEYTADLEDGGWTINIKFAG

SEQ ID NO: 112 - protein, 69 aa, Finegoldia magna
ETPEPEEEVTIKANLIFADGSTQNAEFKGTFAKAVSDAYAYADALKKDNGEYTVDVADKGLTLNIKFAG

SEQ ID NO: 113 - protein, 70 aa, Finegoldia magna
EKPEEPKEEVTIKVNLIFADGKTQTAEFKGTFEEATAKAYAYADLLAKENGEYTADLEDGGNTINIKFAG

SEQ ID NO: 114 - protein, 69 aa, synthetic construct
  REGION 1..69: note = FpL_C1KR
ETPEPEEEVTIRANLIFADGSTQNAEFRGTFARAVSDAYAYADALRRDNGEYTVDVADRGLTLNIRFAG

SEQ ID NO: 115 - protein, 70 aa, synthetic construct
  REGION 1..70: note = FpL_C2KR
ERPEEPREEVTIRVNLIFADGRTQTAEFRGTFEEATARAYAYADLLARENGEYTADLEDGGNTINIRFAG

SEQ ID NO: 116 - protein, 70 aa, synthetic construct
  REGION 1..70: note = FpL_C3KR
ETPEEPREEVTIRVNLIFADGRIQTAEFRGTFEEATARAYAYANLLARENGEYTADLEDGGNTINIRFAG

SEQ ID NO: 117 - protein, 70 aa, synthetic construct
  REGION 1..70: note = FpL_C4KR
ETPEEPREEVTIRVNLIFADGRTQTAEFRGTFEEATAEAYRYADLLARVNGEYTADLEDGGYTINIRFAG

SEQ ID NO: 118 - DNA, 207 bp, synthetic construct
  misc_feature 1..207: note = FpL_C1 DNA
  source 1..207: mol_type = other DNA
gaaactcccgaaccagaggaagaagttacgattaaggctaacttaatcttcgccgacggttcgacacagaatgctgaatttaagggaacattcgcgaaagcggtgtcagatgcatacgcgtacgccgatgcgttgaagaaagataacggtgagtataccgttgacgtagcggataaaggcctgaccttaaatatcaagtttgcgggt

SEQ ID NO: 119 - DNA, 210 bp, synthetic construct
  misc_feature 1..210: note = FpL_C2 DNA
  source 1..210: mol_type = other DNA
gaaaagcccgaagaaccaaaagaagaagttacgattaaggttaacttaatcttcgccgacggtaagacacagacagctgaatttaagggaacattcgaagaagcgaccgcgaaagcatacgcgtacgccgatctgctggcgaaagaaaacggtgagtataccgccgatttagaagatggcggcaatacgatcaatatcaagtttgcgggt

SEQ ID NO: 120 - DNA, 207 bp, synthetic construct
  misc_feature 1..207: note = FpL_C1KR DNA
  source 1..207: mol_type = other DNA
gaaacgccggaaccagaagaggaggttacaattcgcgcgaacttaattttcgcggacggttcgactcagaacgccgaattccgcggtacctttgctcgcgcagtaagcgatgcgtatgcgtacgcagacgccctgcgccgtgataatggcgaatataccgtggatgtcgctgatcgtggcctgaccttgaatatccgttttgccggg

SEQ ID NO: 121 - DNA, 210 bp, synthetic construct
  misc_feature 1..210: note = FpL_C2KR DNA
  source 1..210: mol_type = other DNA
gaacgcccagaagagccgcgcgaagaagttacgatccgtgtgaacttaattttcgcagacggccgtacgcagaccgcggagtttcgtggtacatttgaagaggctaccgcgcgcgcctatgcatatgccgatctgttggctcgcgaaaacggggaatacactgcagatctggaggatggtgggaacaccatcaacattcgtttcgcgggc

SEQ ID NO: 122 - DNA, 210 bp, synthetic construct
  misc_feature 1..210: note = FpL_C3KR DNA
  source 1..210: mol_type = other DNA
gaaaccccagaagaaccgcgcgaggaggtgaccattcgtgttaacttaatctttgcagacggtcgcatccagacagcggaattccgcgggactttcgaagaagcgacagcacgtgcctatgcttatgcgaatttgctggcccgtgaaaacggagaatataccgccgatctggaagatggtggcaatacgatcaacattcgttttgcaggc

SEQ ID NO: 123 - DNA, 210 bp, synthetic construct
  misc_feature 1..210: note = FpL_C4KR DNA
  source 1..210: mol_type = other DNA
gaaacaccagaagagccacgtgaagaagttaccattcgcgtgaatctgatctttgccgacggccgtacccagaccgctgaattccgcggtacattcgaagaagccacagctgaggcctaccgctacgcagatttgctggcgcgcgtcaacggtgaatatacggcggacctggaagatggcgggtataccatcaacatccgctttgcggga

SEQ ID NO: 124 - DNA, 27 bp, synthetic construct
  misc_feature 1..27: note = K7X forward primer 1
  misc_feature 7: note = n is a, c, g, or t
  misc_feature 8: note = d is a, g, or t
  source 1..27: mol_type = other DNA
gagccandtgaagaagttaccattcgc

SEQ ID NO: 125 - DNA, 27 bp, synthetic construct
  misc_feature 1..27: note = K7X forward primer 2
  source 1..27: mol_type = other DNA
gagccavhggaagaagttaccattcgc

SEQ ID NO: 126 - DNA, 27 bp, synthetic construct
  misc_feature 1..27: note = K7X forward primer 3
  source 1..27: mol_type = other DNA
gagccatgggaagaagttaccattcgc

SEQ ID NO: 127 - DNA, 27 bp, synthetic construct
  misc_feature 1..27: note = K7X reverse primer 1
  misc_feature 8: note = h is a, c, or t
  misc_feature 9: note = n is a, c, g, or t
  source 1..27: mol_type = other DNA
ttcttcahntggctcttctggtgtttc

SEQ ID NO: 128 - DNA, 27 bp, synthetic construct
  misc_feature 1..27: note = K7X reverse primer 2
  source 1..27: mol_type = other DNA
ttcttccdbtggctcttctggtgtttc

SEQ ID NO: 129 - DNA, 27 bp, synthetic construct
  misc_feature 1..27: note = K7X reverse primer 3
  source 1..27: mol_type = other DNA
ttcttcccatggctcttctggtgtttc

SEQ ID NO: 130 - DNA, 27 bp, synthetic construct
  misc_feature 1..27: note = K29X forward primer 1
  misc_feature 7: note = n is a, c, g, or t
  misc_feature 8: note = d is a, g, or t
  source 1..27: mol_type = other DNA
gaattcndtggtacattcgaagaagcc

SEQ ID NO: 131 - DNA, 27 bp, synthetic construct
  misc_feature 1..27: note = K29X forward primer 2
  source 1..27: mol_type = other DNA
gaattcvhgggtacattcgaagaagcc

SEQ ID NO: 132 - DNA, 27 bp, synthetic construct
  misc_feature 1..27: note = K29X forward primer 3
  source 1..27: mol_type = other DNA
gaattctggggtacattcgaagaagcc

SEQ ID NO: 133 - DNA, 27 bp, synthetic construct
  misc_feature 1..27: note = K29X reverse primer 1
  misc_feature 8: note = h is a, c, or t
  misc_feature 9: note = n is a, c, g, or t
  source 1..27: mol_type = other DNA
tgtaccahngaattcagcggtctgggt

SEQ ID NO: 134 - DNA, 27 bp, synthetic construct
  misc_feature 1..27: note = K29X reverse primer 2
  source 1..27: mol_type = other DNA
tgtacccdbgaattcagcggtctgggt

SEQ ID NO: 135 - DNA, 27 bp, synthetic construct
  misc_feature 1..27: note = K29X reverse primer 3
  source 1..27: mol_type = other DNA
tgtaccccagaattcagcggtctgggt

SEQ ID NO: 136 - protein, 70 aa, synthetic construct
  REGION 1..70: note = FpL_C4KR K7A
ETPEEPAEEVTIRVNLIFADGRTQTAEFRGTFEEATAEAYRYADLLARVNGEYTADLEDGGYTINIRFAG

SEQ ID NO: 137 - protein, 70 aa, synthetic construct
  REGION 1..70: note = FpL_C4KR K29P
ETPEEPREEVTIRVNLIFADGRTQTAEFPGTFEEATAEAYRYADLLARVNGEYTADLEDGGYTINIRFAG

SEQ ID NO: 138 - protein, 70 aa, synthetic construct
  REGION 1..70: note = FpL_C3KR 1a
ETPEEPREEVTIRVNLIFADRRIQTAEFRGTFEEATARAYAYANLLARENGEYTADLEDGGNTINIRFAG

SEQ ID NO: 139 - protein, 70 aa, synthetic construct
  REGION 1..70: note = FpL_C3KR 1b
ETPEEPREEVTIRVNLIFADGRIQTAEFRGTFEEATARAYAYANLLARENVEYTADLEDGGNTINIRFAG

SEQ ID NO: 140 - protein, 70 aa, synthetic construct
  REGION 1..70: note = FpL_C3KR 1c
ETPEEPREEVTIRVNLIFADGRIQTAEFRGTFEEATARAYAYANLLARENGEYTADLEDGGYTINIRFAG

SEQ ID NO: 141 - protein, 70 aa, synthetic construct
  REGION 1..70: note = FpL_C3KR 3a
ETPEEPREEVTIRVNLIFADGRIQTAEFRGTFEEATARAYAYANLLAREYGGYTADLEDGGYTINIRFAG

SEQ ID NO: 142 - protein, 70 aa, synthetic construct
  REGION 1..70: note = FpL_C3KX
ETPEEPAEEVTIRVNLIFADGQIQTAEFIGTFEEATARAYAYANLLARENGEYTADLEDGGNTINIRFAG

SEQ ID NO: 143 - protein, 70 aa, synthetic construct
  REGION 1..70: note = FpL_C3KX 1a
ETPEEPAEEVTIRVNLIFADRQIQTAEFIGTFEEATARAYAYANLLARENGEYTADLEDGGNTINIRFAG

SEQ ID NO: 144 - protein, 70 aa, synthetic construct
  REGION 1..70: note = FpL_C3KX 3a
ETPEEPAEEVTIRVNLIFADGQIQTAEFIGTFEEATARAYAYANLLAREYGGYTADLEDGGYTINIRFAG

SEQ ID NO: 145 - protein, 70 aa, synthetic construct
  REGION 1..70: note = FpL_C3KX 4g
ETPEEPAEEVTIRVNLIFADRQIQTAEFIGTFEEATARAYAYANLLAREYGGYTADLEDGGYTINIRFAG

SEQ ID NO: 146 - DNA, 27 bp, synthetic construct
  misc_feature 1..27: note = PCR forward primer
  source 1..27: mol_type = other DNA
gcagaccgtcgcatccagacagcggaa

SEQ ID NO: 147 - DNA, 27 bp, synthetic construct
  misc_feature 1..27: note = PCR reverse primer
  source 1..27: mol_type = other DNA
gatgcgacggtctgcaaagattaagtt

SEQ ID NO: 148 - DNA, 27 bp, synthetic construct
  misc_feature 1..27: note = PCR forward primer
  source 1..27: mol_type = other DNA
gaaaacgtggaatatacggcggatctg

SEQ ID NO: 149 - DNA, 27 bp, synthetic construct
  misc_feature 1..27: note = PCR reverse primer
  source 1..27: mol_type = other DNA
atattccacgttttcacgggccagcaa

SEQ ID NO: 150 - DNA, 210 bp, synthetic construct
  misc_feature 1..210: note = FpL_C3KR 1c DNA
  source 1..210: mol_type = other DNA
gaaacaccagaagagccacgtgaagaagttaccattcgcgtgaatctgatctttgccgacggccgtatccagaccgctgaattccgcggtacattcgaagaagccacagctcgtgcctatgcttatgcgaatttgctggcccgtgaaaacggagaatatacggcggacctggaagatggcgggtataccatcaacatccgctttgcggga

SEQ ID NO: 151 - DNA, 24 bp, synthetic construct
  misc_feature 1..24: note = PCR forward primer
  source 1..24: mol_type = other DNA
tatacggcggacctggaagatggc

SEQ ID NO: 152 - DNA, 24 bp, synthetic construct
  misc_feature 1..24: note = PCR reverse primer
  source 1..24: mol_type = other DNA
gtcggcaaagatcagattcacgcg

SEQ ID NO: 153 - DNA, 66 bp, synthetic construct
  misc_feature 1..66: note = Oligonucleotide
  source 1..66: mol_type = other DNA
ctgatctttgccgacggccgtatccagaccgctgaattccgcggtacattcgaagaagccacagct

SEQ ID NO: 154 - DNA, 66 bp, synthetic construct
  misc_feature 1..66: note = Oligonucleotide
  source 1..66: mol_type = other DNA
agctgtggcttcttcgaatgtaccgcggaattcagcggtctggatacggccgtcggcaaagatcag

SEQ ID NO: 155 - DNA, 75 bp, synthetic construct
  misc_feature 1..75: note = Oligonucleotide
  source 1..75: mol_type = other DNA
gaagaagccacagctcgtgcctatgcttatgcgaatttgctggcccgtgaaaacggagaatatacggcggacctg

SEQ ID NO: 156 - DNA, 75 bp, synthetic construct
  misc_feature 1..75: note = Oligonucleotide
  source 1..75: mol_type = other DNA
caggtccgccgtatattctccgttttcacgggccagcaaattcgcataagcataggcacgagctgtggcttcttc

SEQ ID NO: 157 - DNA, 210 bp, synthetic construct
  misc_feature 1..210: note = FpL_C3KR 3a DNA
  source 1..210: mol_type = other DNA
gaaacaccagaagagccacgtgaagaagttaccattcgcgtgaatctgatctttgccgacggccgtatccagaccgctgaattccgcggtacattcgaagaagccacagctcgtgcctatgcttatgcgaatttgctggcccgtgaatatggaggctatacggcggacctggaagatggcgggtataccatcaacatccgctttgcggga

SEQ ID NO: 158 - DNA, 75 bp, synthetic construct
  misc_feature 1..75: note = Oligonucleotide
  source 1..75: mol_type = other DNA
gaagaagccacagctcgtgcctatgcttatgcgaatttgctggcccgtgaatatggaggctatacggcggacctg

SEQ ID NO: 159 - DNA, 75 bp, synthetic construct
  misc_feature 1..75: note = Oligonucleotide
  source 1..75: mol_type = other DNA
caggtccgccgtatagcctccatattcacgggccagcaaattcgcataagcataggcacgagctgtggcttcttc

SEQ ID NO: 160 - DNA, 210 bp, synthetic construct
  misc_feature 1..210: note = FpL_C4KR R7A DNA
  source 1..210: mol_type = other DNA
gaaacaccagaagagccagcggaagaagttaccattcgcgtgaatctgatctttgccgacggccgtacccagaccgctgaattccgcggtacattcgaagaagccacagctgaggcctaccgctacgcagatttgctggcgcgcgtcaacggtgaatatacggcggacctggaagatggcgggtataccatcaacatccgctttgcggga

SEQ ID NO: 161 - DNA, 210 bp, synthetic construct
  misc_feature 1..210: note = FpL_C3KX DNA
  source 1..210: mol_type = other DNA
gaaacaccagaagagccagcggaagaagttaccattcgcgtgaatctgatctttgccgacggccagatccagaccgctgaattcattggtacattcgaagaagccacagctcgtgcctatgcttatgcgaatttgctggcccgtgaaaacggagaatatacggcggacctggaagatggcgggaataccatcaacatccgctttgcggga

SEQ ID NO: 162 - DNA, 36 bp, synthetic construct
  misc_feature 1..36: note = PCR forward primer
  source 1..36: mol_type = other DNA
tatacggcggacctggaagatggcgggaataccatc

SEQ ID NO: 163 - DNA, 66 bp, synthetic construct
  misc_feature 1..66: note = Oligonucleotide
  source 1..66: mol_type = other DNA
ctgatctttgccgacggccagatccagaccgctgaattcattggtacattcgaagaagccacagct

SEQ ID NO: 164 - DNA, 66 bp, synthetic construct
  misc_feature 1..66: note = Oligonucleotide
  source 1..66: mol_type = other DNA
agctgtggcttcttcgaatgtaccaatgaattcagcggtctggatctggccgtcggcaaagatcag

SEQ ID NO: 165 - DNA, 210 bp, synthetic construct
  misc_feature 1..210: note = FpL_C3KX 1a DNA
  source 1..210: mol_type = other DNA
gaaacaccagaagagccagcggaagaagttaccattcgcgtgaatctgatctttgccgaccgccagatccagaccgctgaattcattggtacattcgaagaagccacagctcgtgcctatgcttatgcgaatttgctggcccgtgaaaacggagaatatacggcggacctggaagatggcgggaataccatcaacatccgctttgcggga

SEQ ID NO: 166 - DNA, 66 bp, synthetic construct
  misc_feature 1..66: note = Oligonucleotide
  source 1..66: mol_type = other DNA
ctgatctttgccgaccgccagatccagaccgctgaattcattggtacattcgaagaagccacagct

SEQ ID NO: 167 - DNA, 66 bp, synthetic construct
  misc_feature 1..66: note = Oligonucleotide
  source 1..66: mol_type = other DNA
agctgtggcttcttcgaatgtaccaatgaattcagcggtctggatctggcggtcggcaaagatcag

SEQ ID NO: 168 - DNA, 210 bp, synthetic construct
  misc_feature 1..210: note = FpL_C3KX 3a DNA
  source 1..210: mol_type = other DNA
gaaacaccagaagagccagcggaagaagttaccattcgcgtgaatctgatctttgccgacggtcagattcagaccgctgaattcattggtacattcgaagaagccacagctcgtgcctatgcttatgcgaatttgctggcccgtgaatatggtggctatacggcggacctggaagatggcgggtataccatcaacatccgctttgcggga

SEQ ID NO: 169 - DNA, 66 bp, synthetic construct
  misc_feature 1..66: note = Oligonucleotide
  source 1..66: mol_type = other DNA
ctgatctttgccgacggtcagattcagaccgctgaattcattggtacattcgaagaagccacagct

SEQ ID NO: 170 - DNA, 66 bp, synthetic construct
  misc_feature 1..66: note = Oligonucleotide
  source 1..66: mol_type = other DNA
agctgtggcttcttcgaatgtaccaatgaattcagcggtctgaatctgaccgtcggcaaagatcag

SEQ ID NO: 171 - DNA, 210 bp, synthetic construct
  misc_feature 1..210: note = FpL_C3KX 4g DNA
  source 1..210: mol_type = other DNA
gaaacaccagaagagccagcggaagaagttaccattcgcgtgaatctgatctttgccgaccgtcagattcagaccgctgaattcattggtacattcgaagaagccacagctcgtgcctatgcttatgcgaatttgctggcccgtgaatatggtggctatacggcggacctggaagatggcgggtataccatcaacatccgctttgcggga

SEQ ID NO: 172 - protein, 70 aa, synthetic construct
  REGION 1..70: note = FpL_C3KX 3a E1G
GTPEEPAEEVTIRVNLIFADGQIQTAEFIGTFEEATARAYAYANLLAREYGGYTADLEDGGYTINIRFAG

SEQ ID NO: 173 - protein, 70 aa, synthetic construct
  REGION 1..70: note = FpL_C3KX 3a E1V
VTPEEPAEEVTIRVNLIFADGQIQTAEFIGTFEEATARAYAYANLLAREYGGYTADLEDGGYTINIRFAG

SEQ ID NO: 174 - protein, 70 aa, synthetic construct
  REGION 1..70: note = FpL_C3KX 3a K22R
ETPEEPAEEVTIRVNLIFADGRIQTAEFIGTFEEATARAYAYANLLAREYGGYTADLEDGGYTINIRFAG

SEQ ID NO: 175 - protein, 70 aa, synthetic construct
  REGION 1..70: note = FpL_C3KX 3a E4K
ETPKEPAEEVTIRVNLIFADGQIQTAEFIGTFEEATARAYAYANLLAREYGGYTADLEDGGYTINIRFAG

SEQ ID NO: 176 - protein, 70 aa, synthetic construct
  REGION 1..70: note = FpL_C3KX 3a K22T
ETPEEPAEEVTIRVNLIFADGTIQTAEFIGTFEEATARAYAYANLLAREYGGYTADLEDGGYTINIRFAG

SEQ ID NO: 177 - protein, 70 aa, synthetic construct
  REGION 1..70: note = FpL_C3KX 3a E27R
ETPEEPAEEVTIRVNLIFADGQIQTARFIGTFEEATARAYAYANLLAREYGGYTADLEDGGYTINIRFAG

SEQ ID NO: 178 - protein, 70 aa, synthetic construct
  REGION 1..70: note = FpL_C3KX 3a T36A
ETPEEPAEEVTIRVNLIFADGQIQTAEFIGTFEEAAARAYAYANLLAREYGGYTADLEDGGYTINIRFAG

SEQ ID NO: 179 - protein, 70 aa, synthetic construct
  REGION 1..70: note = FpL_C3KX 4h
ETPEEPAEEVTIRVNLIFADGQIQTAEFIGTFEEATARAYAYANLLARDYGGYTADLEDGGYTINIRFAG

SEQ ID NO: 180 - DNA, 210 bp, synthetic construct
  misc_feature 1..210: note = FpL_C3KX 4h DNA
  source 1..210: mol_type = other DNA
gaaacaccagaagagccagcggaagaagttaccattcgcgtgaatctgatctttgccgacggtcagattcagaccgctgaattcattggtacattcgaagaagccacagctcgtgcctatgcttatgcgaatttgctggcccgtgattatggtggctatacggcggacctggaagatggcgggtataccatcaacatccgctttgcggga

SEQ ID NO: 181 - protein, 70 aa, synthetic construct
  REGION 1..70: note = FpL_C3KX 4h_E9V
ETPEEPAEVVTIRVNLIFADGQIQTAEFIGTFEEATARAYAYANLLARDYGGYTADLEDGGYTINIRFAG

SEQ ID NO: 182 - protein, 70 aa, synthetic construct
  REGION 1..70: note = FpL_C3KX 4i
ETPEEPAEEVTIRVNLIFADGRIQTAEFIGTFEEATARAYAYANLLARDYGGYTADLEDGGYTINIRFAG

SEQ ID NO: 183 - protein, 70 aa, synthetic construct
  REGION 1..70: note = FpL_C3KX 4h Y53F
ETPEEPAEEVTIRVNLIFADGQIQTAEFIGTFEEATARAYAYANLLARDYGGFTADLEDGGYTINIRFAG

SEQ ID NO: 184 - protein, 70 aa, synthetic construct
  REGION 1..70: note = FpL_C3KX 4h T54M
ETPEEPAEEVTIRVNLIFADGQIQTAEFIGTFEEATARAYAYANLLARDYGGYMADLEDGGYTINIRFAG

SEQ ID NO: 185 - protein, 70 aa, synthetic construct
  REGION 1..70: note = FpL_C3KX 4h A69T
ETPEEPAEEVTIRVNLIFADGQIQTAEFIGTFEEATARAYAYANLLARDYGGYTADLEDGGYTINIRFTG

SEQ ID NO: 186 - protein, 70 aa, synthetic construct
  REGION 1..70: note = FpL_C3KX 5e
ETPEEPAEEVTIRVNLIFADGRIQTAEFIGTFEEATARAYAYANLLARDYGGFTADLEDGGYTINIRFAG

SEQ ID NO: 187 - protein, 70 aa, synthetic construct
  REGION 1..70: note = FpL_C3KX 5f
ETPEEPAEEVTIRVNLIFADGRIQTAEFIGTFEEATARAYAYANLLARDYGGYMADLEDGGYTINIRFAG

SEQ ID NO: 188 - DNA, 210 bp, synthetic construct
  misc_feature 1..210: note = FpL_C3KX 4i DNA
  source 1..210: mol_type = other DNA
gaaacaccagaagagccagcggaagaagttaccattcgcgtgaatctgatctttgccgacggtcggattcagaccgctgaattcattggtacattcgaagaagccacagctcgtgcctatgcttatgcgaatttgctggcccgtgattatggtggctatacggcggacctggaagatggcgggtataccatcaacatccgctttgcggga

SEQ ID NO: 189 - DNA, 27 bp, synthetic construct
  misc_feature 1..27: note = PCR forward primer
  source 1..27: mol_type = other DNA
ggtggctttacggcggacctggaagat

SEQ ID NO: 190 - DNA, 27 bp, synthetic construct
  misc_feature 1..27: note = PCR reverse primer
  source 1..27: mol_type = other DNA
cgccgtaaagccaccataatcacgggc

SEQ ID NO: 191 - DNA, 27 bp, synthetic construct
  misc_feature 1..27: note = PCR forward primer
  source 1..27: mol_type = other DNA
ggctatatggcggacctggaagatggc

SEQ ID NO: 192 - DNA, 27 bp, synthetic construct
  misc_feature 1..27: note = PCR reverse primer
  source 1..27: mol_type = other DNA
gtccgccatatagccaccataatcacg

SEQ ID NO: 193 - DNA, 210 bp, synthetic construct
  misc_feature 1..210: note = FpL_C3KX 5e DNA
  source 1..210: mol_type = other DNA
gaaacaccagaagagccagcggaagaagttaccattcgcgtgaatctgatctttgccgacggtcggattcagaccgctgaattcattggtacattcgaagaagccacagctcgtgcctatgcttatgcgaatttgctggcccgtgattatggtggctttacggcggacctggaagatggcgggtataccatcaacatccgctttgcggga

SEQ ID NO: 194 - protein, 70 aa, synthetic construct
  REGION 1..70: note = FpL_C3KX 5e E1V
VTPEEPAEEVTIRVNLIFADGRIQTAEFIGTFEEATARAYAYANLLARDYGGFTADLEDGGYTINIRFAG

SEQ ID NO: 195 - protein, 70 aa, synthetic construct
  REGION 1..70: note = FpL_C3KX 5e E4G
ETPGEPAEEVTIRVNLIFADGRIQTAEFIGTFEEATARAYAYANLLARDYGGFTADLEDGGYTINIRFAG

SEQ ID NO: 196 - protein, 70 aa, synthetic construct
  REGION 1..70: note = FpL_C3KX 5e K7S
ETPEEPSEEVTIRVNLIFADGRIQTAEFIGTFEEATARAYAYANLLARDYGGFTADLEDGGYTINIRFAG

SEQ ID NO: 197 - protein, 70 aa, synthetic construct
  REGION 1..70: note = FpL_C3KX 5e G21R
ETPEEPAEEVTIRVNLIFADRRIQTAEFIGTFEEATARAYAYANLLARDYGGFTADLEDGGYTINIRFAG

SEQ ID NO: 198 - protein, 70 aa, synthetic construct
  REGION 1..70: note = FpL_C3KX 5e G52D
ETPEEPAEEVTIRVNLIFADGRIQTAEFIGTFEEATARAYAYANLLARDYGDFTADLEDGGYTINIRFAG

SEQ ID NO: 199 - protein, 70 aa, synthetic construct
  REGION 1..70: note = FpL_C3KX 6a
ETPGEPAEEVTIRVNLIFADGRIQTAEFIGTFEEATARAYAYANLLARDYGDFTADLEDGGYTINIRFAG

SEQ ID NO: 200 - protein, 70 aa, synthetic construct
  REGION 1..70: note = FpL_C3KX 5g
ETPEEPSEEVTIRVNLIFADGRIQTAEFIGTFEEATARAYAYANLLARDYGDFTADLEDGGYTINIRFAG

SEQ ID NO: 201 - protein, 70 aa, synthetic construct
  REGION 1..70: note = FpL_C3KX 6b
ETPGEPSEEVTIRVNLIFADGRIQTAEFIGTFEEATARAYAYANLLARDYGGFTADLEDGGYTINIRFAG

SEQ ID NO: 202 - DNA, 210 bp, synthetic construct
  misc_feature 1..210: note = FpL_C3KX 5e G52D DNA
  source 1..210: mol_type = other DNA
gaaacaccagaagagccagcggaagaagttaccattcgcgtgaatctgatctttgccgacggtcggattcagaccgctgaattcattggtacattcgaagaagccacagctcgtgcctatgcttatgcgaatttgctggcccgtgattatggtgactttacggcggacctggaagatggcgggtataccatcaacatccgctttgcggga

SEQ ID NO: 203 - DNA, 27 bp, synthetic construct
  misc_feature 1..27: note = PCR forward primer
  source 1..27: mol_type = other DNA
acaccaggagagccagcggaagaagtt

SEQ ID NO: 204 - DNA, 27 bp, synthetic construct
  misc_feature 1..27: note = PCR reverse primer
  source 1..27: mol_type = other DNA
tggctctcctggtgtttccatggtata

SEQ ID NO: 205 - DNA, 27 bp, synthetic construct
  misc_feature 1..27: note = PCR forward primer
  source 1..27: mol_type = other DNA
gagccatcggaagaagttaccattcgc

SEQ ID NO: 206 - DNA, 27 bp, synthetic construct
  misc_feature 1..27: note = PCR reverse primer
  source 1..27: mol_type = other DNA
ttcttccgatggctcttctggtgtttc

SEQ ID NO: 207 - DNA, 210 bp, synthetic construct
  misc_feature 1..210: note = FpL_C3KX 5e E4G DNA
  source 1..210: mol_type = other DNA
gaaacaccaggagagccagcggaagaagttaccattcgcgtgaatctgatctttgccgacggtcggattcagaccgctgaattcattggtacattcgaagaagccacagctcgtgcctatgcttatgcgaatttgctggcccgtgattatggtggctttacggcggacctggaagatggcgggtataccatcaacatccgctttgcggga

SEQ ID NO: 208 - DNA, 27 bp, synthetic construct
  misc_feature 1..27: note = PCR reverse primer
  source 1..27: mol_type = other DNA
ttcttccgatggctctcctggtgtttc

SEQ ID NO: 209 - protein, 719 aa, Finegoldia magna
MAALAGAIVVTGGVGSYAADEPIDLEKLEEKRDKENVGNLPKFDNEVKDGSENPMAKYPDFDDEASTRFETENNEFEEKKVVSDNFFDQSEHPFVENKEETPETPETDSEEEVTIKANLIFANGSTQTAEFKGTFEKATSEAYAYADTLKKDNGEYTVDVADKGYTLNIKFAGKEKTPEEPKEEVTIKANLIYADGKTQTAEFKGTFEEATAEAYRYADALKKDNGEYTVDVADKGYTLNIKFAGKEKTPEEPKEEVTIKANLIYADGKTQTAEFKGTFEEATAEAYRYADLLAKENGKYTVDVADKGYTLNIKFAGKEKTPEEPKEEVTIKANLIYADGKTQTAEFKGTFAEATAEAYRYADLLAKENGKYTADLEDGGYTINIRFAGKKVDEKPEEKEQVTIKENIYFEDGTVQTATFKGTFAEATAEAYRYADLLSKEHGKYTADLEDGGYTINIRFAGKEEPEETPEKPEVQDGYASYEEAEAAAKEALKNDDVNKSYTIRQGADGRYYYVLSPVEAEEEKPEAQNGYATYEEAEAAAKKALENDPINKSYSIRQGADGRYYYVLSPVEAETPEKPVEPSEPSTPDVPSNPSNPSTPDVPSTPDVPSNPSTPEVPSNPSTPGNEEKPGNEQKPGNEQKPGNEQKPGNEQKPGNEQKPDQPSKPEKEENGKGGVDSPKKKEKAALPKAGSEAEILTLAAASLSSVAGAFISLKKRK

SEQ ID NO: 210 - protein, 992 aa, Finegoldia magna
MKINKKLLMAALAGAIVVGGGANAYAAEEDNTDNNLSMDEISDAYFDYHGDVSDSVDPVEEEIDEALAKALAEAKETAKKHIDSLNHLSETAKKLAKNDIDSATTINAINDIVARADVMERKTAEKEEAEKLAAAKETAKKHIDELKHLADKTKELAKRDIDSATTINAINDIVARADVMERKTAEKEEAEKLAAAKETAKKHIDELKHLADKTKELAKRDIDSATTIDAINDIVARADVMERKLSEKETPEPEEEVTIKANLIFADGSTQNAEFKGTFAKAVSDAYAYADALKKDNGEYTVDVADKGLTLNIKFAGKKEKPEEPKEEVTIKVNLIFADGKTQTAEFKGTFEEATAKAYAYADLLAKENGEYTADLEDGGNTINIKFAGKETPETPEEPKEEVTIKVNLIFADGKIQTAEFKGTFEEATAKAYAYANLLAKENGEYTADLEDGGNTINIKFAGKETPETPEEPKEEVTIKVNLIFADGKTQTAEFKGTFEEATAEAYRYADLLAKVNGEYTADLEDGGYTINIKFAGKEQPGENPGITIDEWLLKNAKEEAIKELKEAGITSDLYFSLINKAKTVEGVEALKNEILKAHAGEETPELKDGYATYEEAEAAAKEALKNDDVNNAYEIVQGADGRYYYVLKIEVADEEEPGEDTPEVQEGYATYEEAEAAAKEALKEDKVNNAYEVVQGADGRYYYVLKIEDKEDEQPGEEPGENPGITIDEWLLKNAKEDAIKELKEAGISSDIYFDAINKAKTVEGVEALKNEILKAHAEKPGENPGITIDEWLLKNAKEAAIKELKEAGITAEYLFNLINKAKTVEGVESLKNEILKAHAEKPGENPGITIDEWLLKNAKEDAIKELKEAGITSDIYFDAINKAKTIEGVEALKNEILKAHKKDEEPGKKPGEDKKPEDKKPGEDKKPEDKKPGEDKKPEDKKPGKTDKDSPNKKKKAKLPKAGSEAEILTLAAAALSTAAGAYVSLKKRK

SEQ ID NO: 211 - DNA, 210 bp, synthetic construct
  misc_feature 1..210: note = FpL_C3KX 6a DNA
  source 1..210: mol_type = other DNA
gaaacaccaggagagccagcggaagaagttaccattcgcgtgaatctgatctttgccgacggtcggattcagaccgctgaattcattggtacattcgaagaagccacagctcgtgcctatgcttatgcgaatttgctggcccgtgattatggtgactttacggcggacctggaagatggcgggtataccatcaacatccgctttgcggga

SEQ ID NO: 212 - protein, 70 aa, synthetic construct
  REGION 1..70: note = FpL_C3KX 6a K38A
ETPGEPAEEVTIRVNLIFADGRIQTAEFIGTFEEATAAAYAYANLLARDYGDFTADLEDGGYTINIRFAG

SEQ ID NO: 213 - protein, 70 aa, synthetic construct
  REGION 1..70: note = FpL_C3KX 6a F32L A47T
ETPGEPAEEVTIRVNLIFADGRIQTAEFIGTLEEATARAYAYANLLTRDYGDFTADLEDGGYTINIRFAG

SEQ ID NO: 214 - protein, 70 aa, synthetic construct
  REGION 1..70: note = FpL_C3KX 6a T2S
ESPGEPAEEVTIRVNLIFADGRIQTAEFIGTFEEATARAYAYANLLARDYGDFTADLEDGGYTINIRFAG

SEQ ID NO: 215 - protein, 70 aa, synthetic construct
  REGION 1..70: note = FpL_C3KX 6a E27K
ETPGEPAEEVTIRVNLIFADGRIQTAKFIGTFEEATARAYAYANLLARDYGDFTADLEDGGYTINIRFAG

SEQ ID NO: 216 - protein, 70 aa, synthetic construct
  REGION 1..70: note = FpL_C3KX 6a T2P P3R E9V D52N
EPRGEPAEVVTIRVNLIFADGRIQTAEFIGTFEEATARAYAYANLLARNYGNFTADLEDGGYTINIRFAG

SEQ ID NO: 217 - protein, 70 aa, synthetic construct
  REGION 1..70: note = FpL_C3KX 6a E27I
ETPGEPAEEVTIRVNLIFADGRIQTAIFIGTFEEATARAYAYANLLARDYGDFTADLEDGGYTINIRFAG

SEQ ID NO: 218 - protein, 70 aa, synthetic construct
  REGION 1..70: note = FpL_C3KX 6a N44I
ETPGEPAEEVTIRVNLIFADGRIQTAEFIGTFEEATARAYAYAILLARDYGDFTADLEDGGYTINIRFAG

SEQ ID NO: 219 - protein, 70 aa, synthetic construct
  REGION 1..70: note = FpL_C3KX 6a E5K N44I
ETPGKPAEEVTIRVNLIFADGRIQTAEFIGTFEEATARAYAYAILLARDYGDFTADLEDGGYTINIRFAG

SEQ ID NO: 220 - protein, 70 aa, synthetic construct
  REGION 1..70: note = FpL_C3KX 6a P3R
ETRGEPAEEVTIRVNLIFADGRIQTAEFIGTFEEATARAYAYANLLARDYGDFTADLEDGGYTINIRFAG

SEQ ID NO: 221 - protein, 70 aa, synthetic construct
  REGION 1..70: note = FpL_C3KX 6a E5K
ETPGKPAEEVTIRVNLIFADGRIQTAEFIGTFEEATARAYAYANLLARDYGDFTADLEDGGYTINIRFAG

SEQ ID NO: 222 - protein, 70 aa, synthetic construct
  REGION 1..70: note = FpL_C3KX 6a E27V
ETPGEPAEEVTIRVNLIFADGRIQTAVFIGTFEEATARAYAYANLLARDYGDFTADLEDGGYTINIRFAG

SEQ ID NO: 223 - protein, 70 aa, synthetic construct
  REGION 1..70: note = FpL_C3KX 7a
ETPGRPAEEVTIRVNLIFADGRIQTAEFIGTFEEATARAYAYANLLARDYGDFTADLEDGGYTINIRFAG

SEQ ID NO: 224 - protein, 70 aa, synthetic construct
  REGION 1..70: note = FpL_C3KX 7b
ETPGEPAEEVTIRVNLIFADGRIQTARFIGTFEEATARAYAYANLLARDYGDFTADLEDGGYTINIRFAG

SEQ ID NO: 225 - protein, 70 aa, synthetic construct
  REGION 1..70: note = FpL_C3KX 7c
ETPGEPAEEVTIRVNLIFADGRIQTAEFIGTFEEATARAYAYANLLRRDYGDFTADLEDGGYTINIRFAG

SEQ ID NO: 226 - DNA, 33 bp, synthetic construct
  misc_feature 1..33: note = PCR forward primer
  source 1..33: mol_type = other DNA
gaaacacgaggaagaccagcggaagaagttacc

SEQ ID NO: 227 - DNA, 33 bp, synthetic construct
  misc_feature 1..33: note = PCR reverse primer
  source 1..33: mol_type = other DNA
cgctggtcttcctggtgtttccatggccatcgc

SEQ ID NO: 228 - DNA, 27 bp, synthetic construct
  misc_feature 1..27: note = PCR forward primer
  source 1..27: mol_type = other DNA
accgctagattcattggtacattcgaa

SEQ ID NO: 229 - DNA, 27 bp, synthetic construct
  misc_feature 1..27: note = PCR reverse primer
  source 1..27: mol_type = other DNA
aatgaatctagcggtctgaatccgacc

SEQ ID NO: 230 - DNA, 27 bp, synthetic construct
  misc_feature 1..27: note = PCR forward primer
  source 1..27: mol_type = other DNA
ttgctgaggcgtgattatggtgacttt

SEQ ID NO: 231 - DNA, 27 bp, synthetic construct
  misc_feature 1..27: note = PCR reverse primer
  source 1..27: mol_type = other DNA
atcacgcctcagcaaattcgcataagc

SEQ ID NO: 232 - DNA, 18 bp, synthetic construct
  misc_feature 1..18: note = 6His DNA
  source 1..18: mol_type = other DNA
catcaccaccatcaccac

SEQ ID NO: 233 - DNA, 210 bp, synthetic construct
  misc_feature 1..210: note = FpL_C3KX 5e_DNA
  source 1..210: mol_type = other DNA
gaaacaccagaagagccagcggaagaagttaccattcgcgtgaatctgatctttgccgacggtcggattcagaccgctgaattcattggtacattcgaagaagccacagctcgtgcctatgcttatgcgaatttgctggcccgtgattatggtggctttacggcggacctggaagatggcgggtatacgatcaatatccgttttgcgggc

SEQ ID NO: 234 - DNA, 30 bp, synthetic construct
  misc_feature 1..30: note = PCR forward primer
  source 1..30: mol_type = other DNA
ccagaagagagcgcggaagaagttaccatt

SEQ ID NO: 235 - DNA, 30 bp, synthetic construct
  misc_feature 1..30: note = PCR reverse primer
  source 1..30: mol_type = other DNA
ttcttccgcgctctcttctggtgtttccat

SEQ ID NO: 236 - protein, 70 aa, synthetic construct
  REGION 1..70: note = FpL_C3KX5e_P6S
ETPEESAEEVTIRVNLIFADGRIQTAEFIGTFEEATARAYAYANLLARDYGGFTADLEDGGYTINIRFAG

SEQ ID NO: 237 - DNA, 27 bp, synthetic construct
  misc_feature 1..27: note = PCR forward primer
  source 1..27: mol_type = other DNA
acagcagaagcctatgcttatgcgaat

SEQ ID NO: 238 - DNA, 27 bp, synthetic construct
  misc_feature 1..27: note = PCR reverse primer
  source 1..27: mol_type = other DNA
ataggcttctgctgtcgcttcttcgaa

SEQ ID NO: 239 - protein, 70 aa, synthetic construct
  REGION 1..70: note = FpL_C3KR_K38E
ETPEEPREEVTIRVNLIFADGRIQTAEFRGTFEEATAEAYAYANLLARENGEYTADLEDGGNTINIRFAG

SEQ ID NO: 240 - protein, 70 aa, synthetic construct
  REGION 1..70: note = FpL_C3KX 7d
ETPGESAEEVTIRVNLIFADGRIQTAEFIGTFEEATAEAYAYANLLARDYGDFTADLEDGGYTINIRFAG

SEQ ID NO: 241 - DNA, 210 bp, synthetic construct
  misc_feature 1..210: note = FpL_C3KX 7d_DNA
  source 1..210: mol_type = other DNA
gaaacaccaggagagtcagcggaagaagttaccattcgcgtgaatctgatctttgccgacggtcggattcagaccgctgaattcattggtacattcgaagaagccacagctgaagcctatgcttatgcgaatttgctggcccgtgattatggtgactttacggcggacctggaagatggcgggtataccatcaacatccgctttgcggga

SEQ ID NO: 242 - protein, 70 aa, synthetic construct
  REGION 1..70: note = FpL_C3KX 7d_A69V
ETPGESAEEVTIRVNLIFADGRIQTAEFIGTFEEATAEAYAYANLLARDYGDFTADLEDGGYTINIRFVG

SEQ ID NO: 243 - protein, 70 aa, synthetic construct
  REGION 1..70: note = FpL_C3KX 7d_I29F
ETPGESAEEVTIRVNLIFADGRIQTAEFFGTFEEATAEAYAYANLLARDYGDFTADLEDGGYTINIRFAG

SEQ ID NO: 244 - protein, 70 aa, synthetic construct
  REGION 1..70: note = FpL_C3KX 7d_E8G,E33V
ETPGESAGEVTIRVNLIFADGRIQTAEFIGTFVEATAEAYAYANLLARDYGDFTADLEDGGYTINIRFAG

SEQ ID NO: 245 - DNA, 27 bp, synthetic construct
  misc_feature 1..27: note = I23X forward primer 1
  misc_feature 7: note = n is a, c, g, or t
  source 1..27: mol_type = other DNA
ggtcggndtcagaccgctgaattcatt

SEQ ID NO: 246 - DNA, 27 bp, synthetic construct
  misc_feature 1..27: note = I23X forward primer 2
  source 1..27: mol_type = other DNA
ggtcggvhgcagaccgctgaattcatt

SEQ ID NO: 247 - DNA, 27 bp, synthetic construct
  misc_feature 1..27: note = I23X forward primer 3
  source 1..27: mol_type = other DNA
ggtcggtggcagaccgctgaattcatt

SEQ ID NO: 248 - DNA, 27 bp, synthetic construct
  misc_feature 1..27: note = I23X reverse primer 1
  misc_feature 9: note = n is a, c, g, or t
  source 1..27: mol_type = other DNA
accgtcahnccgaccgtcggcaaagat

SEQ ID NO: 249 - DNA, 27 bp, synthetic construct
  misc_feature 1..27: note = I23X reverse primer 2
  source 1..27: mol_type = other DNA
accgtccdbccgaccgtcggcaaagat

SEQ ID NO: 250 - DNA, 27 bp, synthetic construct
  misc_feature 1..27: note = A41X forward primer 1
  source 1..27: mol_type = other DNA
accgtcccaccgaccgtcggcaaagat

SEQ ID NO: 251 - protein, 70 aa, synthetic construct
  REGION 1..70: note = FpL_C3KX 7d_I23R
ETPGESAEEVTIRVNLIFADGRRQTAEFIGTFEEATAEAYAYANLLARDYGDFTADLEDGGYTINIRFAG

SEQ ID NO: 252 - DNA, 27 bp, synthetic construct
  misc_feature 1..27: note = A41X forward primer 1
  misc_feature 7: note = n is a, c, g, or t
  source 1..27: mol_type = other DNA
gcctatndttatgcgaatttgctggcc

SEQ ID NO: 253 - DNA, 27 bp, synthetic construct
  misc_feature 1..27: note = A41X forward primer 2
  source 1..27: mol_type = other DNA
gcctatvhgtatgcgaatttgctggcc

SEQ ID NO: 254 - DNA, 27 bp, synthetic construct
  misc_feature 1..27: note = A41X forward primer 3
  source 1..27: mol_type = other DNA
gcctattggtatgcgaatttgctggcc

SEQ ID NO: 255 - DNA, 27 bp, synthetic construct
  misc_feature 1..27: note = A41X reverse primer 1
  misc_feature 9: note = n is a, c, g, or t
  source 1..27: mol_type = other DNA
ggcttcahnataggcttcagctgtggc

SEQ ID NO: 256 - DNA, 27 bp, synthetic construct
  misc_feature 1..27: note = A41X reverse primer 2
  source 1..27: mol_type = other DNA
ggcttccdbataggcttcagctgtggc

SEQ ID NO: 257 - DNA, 27 bp, synthetic construct
  misc_feature 1..27: note = A41X reverse primer 3
  source 1..27: mol_type = other DNA
ggcttcccaataggcttcagctgtggc

SEQ ID NO: 258 - protein, 70 aa, synthetic construct
  REGION 1..70: note = FpL_C3KX 7d_A41I
ETPGESAEEVTIRVNLIFADGRIQTAEFIGTFEEATAEAYIYANLLARDYGDFTADLEDGGYTINIRFAG

SEQ ID NO: 259 - protein, 70 aa, synthetic construct
  REGION 1..70: note = FpL_C3KX 7d_A41Y
ETPGESAEEVTIRVNLIFADGRIQTAEFIGTFEEATAEAYYYANLLARDYGDFTADLEDGGYTINIRFAG

SEQ ID NO: 260 - DNA, 27 bp, synthetic construct
  misc_feature 1..27: note = E52X forward primer 1
  misc_feature 7: note = n is a, c, g, or t
  source 1..27: mol_type = other DNA
tatggtndttttacggcggacctggaa

SEQ ID NO: 261 - DNA, 27 bp, synthetic construct
  misc_feature 1..27: note = E52X forward primer 2
  source 1..27: mol_type = other DNA
tatggtvhgtttacggcggacctggaa

SEQ ID NO: 262 - DNA, 27 bp, synthetic construct
  misc_feature 1..27: note = E52X forward primer 3
  source 1..27: mol_type = other DNA
tatggttggtttacggcggacctggaa

SEQ ID NO: 263 - DNA, 27 bp, synthetic construct
  misc_feature 1..27: note = E52X reverse primer 1
  misc_feature 9: note = n is a, c, g, or t
  source 1..27: mol_type = other DNA
ataatcahnaccataatcacgggccag

SEQ ID NO: 264 - DNA, 27 bp, synthetic construct
  misc_feature 1..27: note = E52X reverse primer 2
  source 1..27: mol_type = other DNA
ataatccdbaccataatcacgggccag

SEQ ID NO: 265 - DNA, 27 bp, synthetic construct
  misc_feature 1..27: note = E52X reverse primer 3
  source 1..27: mol_type = other DNA
ataatcccaaccataatcacgggccag

SEQ ID NO: 266 - protein, 70 aa, synthetic construct
  REGION 1..70: note = FpL_C3KX 7d_E52L
ETPGESAEEVTIRVNLIFADGRIQTAEFIGTFEEATAEAYAYANLLARDYGLFTADLEDGGYTINIRFAG

SEQ ID NO: 267 - protein, 70 aa, synthetic construct
  REGION 1..70: note = FpL_C3KX 7d_E52V
ETPGESAEEVTIRVNLIFADGRIQTAEFIGTFEEATAEAYAYANLLARDYGVFTADLEDGGYTINIRFAG

SEQ ID NO: 268 - DNA, 210 bp, synthetic construct
  misc_feature 1..210: note = FpL_C3KX 7d_A69V_DNA
  source 1..210: mol_type = other DNA
gaaacaccaggagagtcagcggaagaagttaccattcgcgtgaatctgatctttgccgacggtcggattcagaccgccgaattcattggtacattcgaagaagccacagctgaagcctatgcttatgcgaatttgctggcccgtgattatggtgactttacggcggacctggaagatggcgggtataccatcaacatccgctttgtggga

SEQ ID NO: 269 - DNA, 30 bp, synthetic construct
  misc_feature 1..30: note = PCR forward primer
  source 1..30: mol_type = other DNA
gattatggtgtgtttacggcggacctggaa

SEQ ID NO: 270 - DNA, 30 bp, synthetic construct
  misc_feature 1..30: note = PCR reverse primer
  source 1..30: mol_type = other DNA
cgccgtaaacacaccataatcacgggccag

SEQ ID NO: 271 - protein, 70 aa, synthetic construct
  REGION 1..70: note = FpL_C3KX 8a
ETPGESAEEVTIRVNLIFADGRIQTAEFIGTFEEATAEAYAYANLLARDYGVFTADLEDGGYTINIRFVG

SEQ ID NO: 272 - DNA, 30 bp, synthetic construct
  misc_feature 1..30: note = PCR forward primer
  source 1..30: mol_type = other DNA
gattatggtctgtttacggcggacctggaa

SEQ ID NO: 273 - DNA, 30 bp, synthetic construct
  misc_feature 1..30: note = PCR reverse primer
  source 1..30: mol_type = other DNA
cgccgtaaacagaccataatcacgggccag

SEQ ID NO: 274 - protein, 70 aa, synthetic construct
  REGION 1..70: note = FpL_C3KX 8b
ETPGESAEEVTIRVNLIFADGRIQTAEFIGTFEEATAEAYAYANLLARDYGLFTADLEDGGYTINIRFVG

SEQ ID NO: 275 - protein, 70 aa, synthetic construct
  REGION 1..70: note = FpL_C3KX 7e
ETPGESAEEVTIRVNLIFADGRIQTAEFIGTFEEATAEAYAYANLLARDYGEFTADLEDGGYTINIRFVG

SEQ ID NO: 276 - DNA, 210 bp, synthetic construct
  misc_feature 1..210: note = FpL_C3KX 7e_DNA
  source 1..210: mol_type = other DNA
gaaaccccgggagaatcggctgaagaggtcaccattcgtgtgaacttaatcttcgctgatggtcgcatccaaacggcagagttcattgggacgtttgaagaagcaaccgccgaagcgtacgcgtacgccaacctcctcgcccgcgattacggtgaatttacagccgatttggaagatggcggttatacgatcaatatccgcttcgtgggc

SEQ ID NO: 277 - DNA, 30 bp, synthetic construct
  misc_feature 1..30: note = PCR forward primer
  source 1..30: mol_type = other DNA
gattatggtgaatttacggcggacctggaa

SEQ ID NO: 278 - DNA, 30 bp, synthetic construct
  misc_feature 1..30: note = PCR reverse primer
  source 1..30: mol_type = other DNA
cgccgtaaattcaccataatcacgggccag

SEQ ID NO: 279 - protein, 70 aa, synthetic construct
  REGION 1..70: note = FpL_C3KX 7e_P3R
ETRGESAEEVTIRVNLIFADGRIQTAEFIGTFEEATAEAYAYANLLARDYGEFTADLEDGGYTINIRFVG

SEQ ID NO: 280 - protein, 70 aa, synthetic construct
  REGION 1..70: note = FpL_C3KX 7e_P3R,K38R
ETRGESAEEVTIRVNLIFADGRIQTAEFIGTFEEATARAYAYANLLARDYGEFTADLEDGGYTINIRFVG

SEQ ID NO: 281 - protein, 70 aa, synthetic construct
  REGION 1..70: note = FpL_C3KX 7e_P3R,I66V
ETRGESAEEVTIRVNLIFADGRIQTAEFIGTFEEATAEAYAYANLLARDYGEFTADLEDGGYTINVRFVG

SEQ ID NO: 282 - protein, 70 aa, synthetic construct
  REGION 1..70: note = FpL_C3KX 7e_P3R,T31M
ETRGESAEEVTIRVNLIFADGRIQTAEFIGMFEEATAEAYAYANLLARDYGEFTADLEDGGYTINIRFVG

SEQ ID NO: 283 - protein, 70 aa, synthetic construct
  REGION 1..70: note = FpL_C3KX 7e_P6L
ETPGELAEEVTIRVNLIFADGRIQTAEFIGTFEEATAEAYAYANLLARDYGEFTADLEDGGYTINIRFVG

SEQ ID NO: 284 - protein, 70 aa, synthetic construct
  REGION 1..70: note = FpL_C3KX 7e_A35T
ETPGESAEEVTIRVNLIFADGRIQTAEFIGTFEETTAEAYAYANLLARDYGEFTADLEDGGYTINIRFVG

SEQ ID NO: 285 - protein, 70 aa, synthetic construct
  REGION 1..70: note = FpL_C3KX 7e_E33G
ETPGESAEEVTIRVNLIFADGRIQTAEFIGTFGEATAEAYAYANLLARDYGEFTADLEDGGYTINIRFVG

SEQ ID NO: 286 - protein, 70 aa, synthetic construct
  REGION 1..70: note = FpL_C3KX 7e_E5D,P6L
ETPGDLAEEVTIRVNLIFADGRIQTAEFIGTFEEATAEAYAYANLLARDYGEFTADLEDGGYTINIRFVG

SEQ ID NO: 287 - protein, 70 aa, synthetic construct
  REGION 1..70: note = FpL_C3KX 7e_A69L
ETPGESAEEVTIRVNLIFADGRIQTAEFIGTFEEATAEAYAYANLLARDYGEFTADLEDGGYTINIRFLG

SEQ ID NO: 288 - protein, 70 aa, synthetic construct
  REGION 1..70: note = FpL_C3KX 7e_A37T
ETPGESAEEVTIRVNLIFADGRIQTAEFIGTFEEATTEAYAYANLLARDYGEFTADLEDGGYTINIRFVG

SEQ ID NO: 289 - protein, 70 aa, synthetic construct
  REGION 1..70: note = FpL_C3KX 7e_E33D,E52G
ETPGESAEEVTIRVNLIFADGRIQTAEFIGTFDEATAEAYAYANLLARDYGGFTADLEDGGYTINIRFVG

SEQ ID NO: 290 - protein, 70 aa, synthetic construct
  REGION 1..70: note = FpL_C3KX 7e_T2A,K7P
EAPGESPEEVTIRVNLIFADGRIQTAEFIGTFEEATAEAYAYANLLARDYGEFTADLEDGGYTINIRFVG

SEQ ID NO: 291 - protein, 70 aa, synthetic construct
  REGION 1..70: note = FpL_C3KX 7e_I23V
ETPGESAEEVTIRVNLIFADGRVQTAEFIGTFEEATAEAYAYANLLARDYGEFTADLEDGGYTINIRFVG

SEQ ID NO: 292 - protein, 70 aa, synthetic construct
  REGION 1..70: note = FpL_C3KX 7e_P6T
ETPGETAEEVTIRVNLIFADGRIQTAEFIGTFEEATAEAYAYANLLARDYGEFTADLEDGGYTINIRFVG

SEQ ID NO: 293 - protein, 70 aa, synthetic construct
  REGION 1..70: note = FpL_C3KX 7e_T36S
ETPGESAEEVTIRVNLIFADGRIQTAEFIGTFEEASAEAYAYANLLARDYGEFTADLEDGGYTINIRFVG

SEQ ID NO: 294 - DNA, 30 bp, synthetic construct
  misc_feature 1..30: note = PCR forward primer
  source 1..30: mol_type = other DNA
accattcgtgcgaacttaatcttcgctgat

SEQ ID NO: 295 - DNA, 30 bp, synthetic construct
  misc_feature 1..30: note = PCR reverse primer
  source 1..30: mol_type = other DNA
gattaagttcgcacgaatggtgacctcttc

SEQ ID NO: 296 - protein, 70 aa, synthetic construct
  REGION 1..70: note = FpL_C3KX 7e_V14A
ETPGESAEEVTIRANLIFADGRIQTAEFIGTFEEATAEAYAYANLLARDYGEFTADLEDGGYTINIRFVG

SEQ ID NO: 297 - DNA, 30 bp, synthetic construct
  misc_feature 1..30: note = PCR forward primer
  source 1..30: mol_type = other DNA
ttcgctgatcgtcgcatccaaacggcagag

SEQ ID NO: 298 - DNA, 30 bp, synthetic construct
  misc_feature 1..30: note = PCR reverse primer
  source 1..30: mol_type = other DNA
ttggatgcgacgatcagcgaagattaagtt

SEQ ID NO: 299 - protein, 70 aa, synthetic construct
  REGION 1..70: note = FpL_C3KX 7e_G21R
ETPGESAEEVTIRVNLIFADRRIQTAEFIGTFEEATAEAYAYANLLARDYGEFTADLEDGGYTINIRFVG

SEQ ID NO: 300 - DNA, 30 bp, synthetic construct
  misc_feature 1..30: note = PCR forward primer
  source 1..30: mol_type = other DNA
gatggtcgcacccaaacggcagagttcatt

SEQ ID NO: 301 - DNA, 30 bp, synthetic construct
  misc_feature 1..30: note = PCR reverse primer
  source 1..30: mol_type = other DNA
tgccgtttgggtgcgaccatcagcgaagat

SEQ ID NO: 302 - protein, 70 aa, synthetic construct
  REGION 1..70: note = FpL_C3KX 7e_I23T
ETPGESAEEVTIRVNLIFADGRTQTAEFIGTFEEATAEAYAYANLLARDYGEFTADLEDGGYTINIRFVG

SEQ ID NO: 303 - DNA, 30 bp, synthetic construct
  misc_feature 1..30: note = PCR forward primer
  source 1..30: mol_type = other DNA
gaagcgtaccgttacgccaacctcctcgcc

SEQ ID NO: 304 - DNA, 30 bp, synthetic construct
  misc_feature 1..30: note = PCR reverse primer
  source 1..30: mol_type = other DNA
gttggcgtaacggtacgcttcggcggttgc

SEQ ID NO: 305 - protein, 70 aa, synthetic construct
  REGION 1..70: note = FpL_C3KX 7e_A41R
ETPGESAEEVTIRVNLIFADGRIQTAEFIGTFEEATAEAYRYANLLARDYGEFTADLEDGGYTINIRFVG

SEQ ID NO: 306 - DNA, 30 bp, synthetic construct
  misc_feature 1..30: note = PCR forward primer
  source 1..30: mol_type = other DNA
gcgtacgccgatctcctcgcccgcgattac

SEQ ID NO: 307 - DNA, 30 bp, synthetic construct
  misc_feature 1..30: note = PCR reverse primer
  source 1..30: mol_type = other DNA
ggcgaggagatcggcgtacgcgtacgcttc

SEQ ID NO: 308 - protein, 70 aa, synthetic construct
  REGION 1..70: note = FpL_C3KX 7e_N44D
ETPGESAEEVTIRVNLIFADGRIQTAEFIGTFEEATAEAYAYADLLARDYGEFTADLEDGGYTINIRFVG

SEQ ID NO: 309 - DNA, 30 bp, synthetic construct
  misc_feature 1..30: note = PCR forward primer
  source 1..30: mol_type = other DNA
gcgtacgcccgtctcctcgcccgcgattac

SEQ ID NO: 310 - DNA, 30 bp, synthetic construct
  misc_feature 1..30: note = PCR reverse primer
  source 1..30: mol_type = other DNA
ggcgaggagacgggcgtacgcgtacgcttc

SEQ ID NO: 311 - protein, 70 aa, synthetic construct
  REGION 1..70: note = FpL_C3KX 7e_N44R
ETPGESAEEVTIRVNLIFADGRIQTAEFIGTFEEATAEAYAYARLLARDYGEFTADLEDGGYTINIRFVG

SEQ ID NO: 312 - DNA, 30 bp, synthetic construct
  misc_feature 1..30: note = PCR forward primer
  source 1..30: mol_type = other DNA
gcgtacgcccatctcctcgcccgcgattac

SEQ ID NO: 313 - DNA, 30 bp, synthetic construct
  misc_feature 1..30: note = PCR reverse primer
  source 1..30: mol_type = other DNA
ggcgaggagatgggcgtacgcgtacgcttc

SEQ ID NO: 314 - protein, 70 aa, synthetic construct
  REGION 1..70: note = FpL_C3KX 7e_N44H
ETPGESAEEVTIRVNLIFADGRIQTAEFIGTFEEATAEAYAYAHLLARDYGEFTADLEDGGYTINIRFVG

SEQ ID NO: 315 - DNA, 30 bp, synthetic construct
  misc_feature 1..30: note = PCR forward primer
  source 1..30: mol_type = other DNA
gattacggttattttacagccgatttggaa

SEQ ID NO: 316 - DNA, 30 bp, synthetic construct
  misc_feature 1..30: note = PCR reverse primer
  source 1..30: mol_type = other DNA
ggctgtaaaataaccgtaatcgcgggcgag

SEQ ID NO: 317 - protein, 70 aa, synthetic construct
  REGION 1..70: note = FpL_C3KX 7e_E52Y
ETPGESAEEVTIRVNLIFADGRIQTAEFIGTFEEATAEAYAYANLLARDYGYFTADLEDGGYTINIRFVG

SEQ ID NO: 318 - DNA, 30 bp, synthetic construct
  misc_feature 1..30: note = PCR forward primer
  source 1..30: mol_type = other DNA
ttggaagatcgtggttatacgatcaatatc

SEQ ID NO: 319 - DNA, 30 bp, synthetic construct
  misc_feature 1..30: note = PCR reverse primer
  source 1..30: mol_type = other DNA
cgtataaccacgatcttccaaatcggctgt

SEQ ID NO: 320 - protein, 70 aa, synthetic construct
  REGION 1..70: note = FpL_C3KX 7e_G60R
ETPGESAEEVTIRVNLIFADGRIQTAEFIGTFEEATAEAYAYANLLARDYGEFTADLEDRGYTINIRFVG

SEQ ID NO: 321 - DNA, 30 bp, synthetic construct
  misc_feature 1..30: note = PCR forward primer
  source 1..30: mol_type = other DNA
ggttatacgctgaatatccgcttcgtgggc

SEQ ID NO: 322 - DNA, 30 bp, synthetic construct
  misc_feature 1..30: note = PCR reverse primer
  source 1..30: mol_type = other DNA
gcggatattcagcgtataaccgccatcttc

SEQ ID NO: 323 - protein, 70 aa, synthetic construct
  REGION 1..70: note = FpL_C3KX 7e_I64L
ETPGESAEEVTIRVNLIFADGRIQTAEFIGTFEEATAEAYAYANLLARDYGEFTADLEDGGYTLNIRFVG

SEQ ID NO: 324 - protein, 23 aa, synthetic construct
  REGION 1..23: note = Immobilization tag (IT)
ALPSKSKKILKEAKKLNKAQAPK

SEQ ID NO: 325 - protein, 6 aa, synthetic construct
  REGION 1..6: note = 6-Histidine tag (6H)
HHHHHH

SEQ ID NO: 326 - protein, 312 aa, synthetic construct
  REGION 1..312: note = (FpL_C3KX 7e)4-IT-6H3K
ETPGESAEEVTIRVNLIFADGRIQTAEFIGTFEEATAEAYAYANLLARDYGEFTADLEDGGYTINIRFVGETPGESAEEVTIRVNLIFADGRIQTAEFIGTFEEATAEAYAYANLLARDYGEFTADLEDGGYTINIRFVGETPGESAEEVTIRVNLIFADGRIQTAEFIGTFEEATAEAYAYANLLARDYGEFTADLEDGGYTINIRFVGETPGESAEEVTIRVNLIFADGRIQTAEFIGTFEEATAEAYAYANLLARDYGEFTADLEDGGYTINIRFVGALPSKSKKILKEAKKLNKAQAPKHHHHHHKKK

SEQ ID NO: 327 - DNA, 939 bp, synthetic construct
  misc_feature 1..939: note = (FpL_C3KX 7e)4-IT-6H3K_DNA
  source 1..939: mol_type = other DNA
gaaaccccgggagaatcggctgaagaggtcaccattcgtgtgaacttaatcttcgctgatggtcgcatccaaacggcagagttcattgggacgtttgaagaagcaaccgccgaagcgtacgcgtacgccaacctcctcgcccgcgattacggtgaatttacagccgatttggaagatggcggttatacgattaatattcgtttcgttggggaaaccccgggagaatcggctgaagaggtcaccattcgtgtgaacttaatcttcgctgatggtcgcatccaaacggcagagttcattgggacgtttgaagaagcaaccgccgaagcgtacgcgtacgccaacctcctcgcccgcgattacggtgaatttacagccgatttggaagatggcggttatacgatcaatatccgcttcgtgggcgagaccccgggcgaatcggccgaggaggtcaccattcgtgtgaacttaatcttcgctgatggtcgcatccaaacggcagagttcattgggacgtttgaagaagcaaccgccgaagcgtacgcgtacgccaacctcctcgcccgcgattacggtgaatttacagccgatttggaagatggcggttatactatcaatatccgcttcgtcggcgaaaccccgggagaatcggctgaagaggtcaccattcgtgtgaacttaatcttcgctgatggtcgcatccaaacggcagagttcattgggacgtttgaagaagcaaccgccgaagcgtacgcgtacgccaacctcctcgcccgcgattacggtgaatttacagccgatttggaagatggcggttatacgatcaatatccgcttcgtgggcgcgctgccgtctaaatcgaagaaaattctgaaagaagccaagaaactgaataaagctcaggcgccgaaacatcaccaccatcaccacaagaagaaataa

SEQ ID NO: 328 - DNA, 69 bp, synthetic construct
  misc_feature 1..69: note = Immobilization tag_DNA
  source 1..69: mol_type = other DNA
gcgctgccgtctaaatcgaagaaaattctgaaagaagccaagaaactgaataaagctcaggcgccgaaa

SEQ ID NO: 329 - DNA, 51 bp, synthetic construct
  misc_feature 1..51: note = PCR forward primer
  source 1..51: mol_type = other DNA
ctcgctgcccagccggcgatggccatggaaaccccgggagaatcggctgaa

SEQ ID NO: 330 - DNA, 48 bp, synthetic construct
  misc_feature 1..48: note = PCR reverse primer
  source 1..48: mol_type = other DNA
cccaacgaaacgaatattaatcgtataaccgccatcttccaaatcggc

SEQ ID NO: 331 - DNA, 48 bp, synthetic construct
  misc_feature 1..48: note = PCR forward primer
  source 1..48: mol_type = other DNA
acgattaatattcgtttcgttggggaaaccccgggagaatcggctgaa

SEQ ID NO: 332 - DNA, 48 bp, synthetic construct
  misc_feature 1..48: note = PCR reverse primer
  source 1..48: mol_type = other DNA
ctcggccgattcgcccggggtctcgcccacgaagcggatattgatcgt

SEQ ID NO: 333 - DNA, 48 bp, synthetic construct
  misc_feature 1..48: note = PCR forward primer
  source 1..48: mol_type = other DNA
gagaccccgggcgaatcggccgaggaggtcaccattcgtgtgaactta

SEQ ID NO: 334 - DNA, 48 bp, synthetic construct
  misc_feature 1..48: note = PCR reverse primer
  source 1..48: mol_type = other DNA
gccgacgaagcggatattgatagtataaccgccatcttccaaatcggc

SEQ ID NO: 335 - DNA, 48 bp, synthetic construct
  misc_feature 1..48: note = PCR forward primer
  source 1..48: mol_type = other DNA
actatcaatatccgcttcgtcggcgaaaccccgggagaatcggctgaa

SEQ ID NO: 336 - DNA, 78 bp, synthetic construct
  misc_feature 1..78: note = PCR reverse primer
  source 1..78: mol_type = other DNA
tttattcagtttcttggcttctttcagaattttcttcgatttagacggcagcgcgcccacgaagcggatattgatcgt

SEQ ID NO: 337 - DNA, 69 bp, synthetic construct
  misc_feature 1..69: note = Oligonucleotide
  source 1..69: mol_type = other DNA
aaagaagccaagaaactgaataaagctcaggcgccgaaacatcaccaccatcaccacaagaagaaataa

SEQ ID NO: 338 - DNA, 69 bp, synthetic construct
  misc_feature 1..69: note = Oligonucleotide
  source 1..69: mol_type = other DNA
ttatttcttcttgtggtgatggtggtgatgtttcggcgcctgagctttattcagtttcttggcttcttt

SEQ ID NO: 339 - DNA, 42 bp, synthetic construct
  misc_feature 1..42: note = PCR forward primer
  source 1..42: mol_type = other DNA
caccatcaccacaagaagaaataagcttgcggccgcactcga

SEQ ID NO: 340 - DNA, 27 bp, synthetic construct
  misc_feature 1..27: note = PCR reverse primer
  source 1..27: mol_type = other DNA
catggccatcgccggctgggcagcgag

SEQ ID NO: 341 - protein, 70 aa, synthetic construct
  REGION 1..70: note = FpL_C3KX 6c
ETPGESAEEVTIRVNLIFADGRIQTAEFIGTFEEATAEAYAYANLLARDNGEFTADLEDGGYTINIRFVG

SEQ ID NO: 342 - DNA, 210 bp, synthetic construct
  misc_feature 1..210: note = FpL_C3KX 6c_DNA
  source 1..210: mol_type = other DNA
gaaaccccgggagaatcggctgaagaggtcaccattcgtgtgaacttaatcttcgctgatggtcgcatccaaacggcagagttcattgggacgtttgaagaagcaaccgccgaagcgtacgcgtacgccaacctcctcgcccgcgataacggtgaatttacagccgatttggaagatggcggttatacgatcaatatccgcttcgtgggc

SEQ ID NO: 343 - protein, 312 aa, synthetic construct
  REGION 1..312: note = (FpL_C3KX 6c)4-IT-6H3K
ETPGESAEEVTIRVNLIFADGRIQTAEFIGTFEEATAEAYAYANLLARDNGEFTADLEDGGYTINIRFVGETPGESAEEVTIRVNLIFADGRIQTAEFIGTFEEATAEAYAYANLLARDNGEFTADLEDGGYTINIRFVGETPGESAEEVTIRVNLIFADGRIQTAEFIGTFEEATAEAYAYANLLARDNGEFTADLEDGGYTINIRFVGETPGESAEEVTIRVNLIFADGRIQTAEFIGTFEEATAEAYAYANLLARDNGEFTADLEDGGYTINIRFVGALPSKSKKILKEAKKLNKAQAPKHHHHHHKKK

SEQ ID NO: 344 - DNA, 939 bp, synthetic construct
  misc_feature 1..939: note = (FpL_C3KX 6c)4-IT-6H3K_DNA
  source 1..939: mol_type = other DNA
gaaaccccgggagaatcggctgaagaggtcaccattcgtgtgaacttaatcttcgctgatggtcgcatccaaacggcagagttcattgggacgtttgaagaagcaaccgccgaagcgtacgcgtacgccaacctcctcgcccgcgataacggtgaatttacagccgatttggaagatggcggttatacgattaatattcgtttcgttggggaaaccccgggagaatcggctgaagaggtcaccattcgtgtgaacttaatcttcgctgatggtcgcatccaaacggcagagttcattgggacgtttgaagaagcaaccgccgaagcgtacgcgtacgccaacctcctcgcccgcgataacggtgaatttacagccgatttggaagatggcggttatacgatcaatatccgcttcgtgggcgagaccccgggcgaatcggccgaggaggtcaccattcgtgtgaacttaatcttcgctgatggtcgcatccaaacggcagagttcattgggacgtttgaagaagcaaccgccgaagcgtacgcgtacgccaacctcctcgcccgcgataacggtgaatttacagccgatttggaagatggcggttatactatcaatatccgcttcgtcggcgaaaccccgggagaatcggctgaagaggtcaccattcgtgtgaacttaatcttcgctgatggtcgcatccaaacggcagagttcattgggacgtttgaagaagcaaccgccgaagcgtacgcgtacgccaacctcctcgcccgcgataacggtgaatttacagccgatttggaagatggcggttatacgatcaatatccgcttcgtgggcgcgctgccgtctaaatcgaagaaaattctgaaagaagccaagaaactgaataaagctcaggcgccgaaacatcaccaccatcaccacaagaagaaataa

SEQ ID NO: 345 - DNA, 27 bp, synthetic construct
  misc_feature 1..27: note = K13X forward primer 1
  misc_feature 7: note = n is a, c, g, or t
  misc_feature 8: note = d is a, g, or t
  source 1..27: mol_type = other DNA
accattndtgtgaatctgatctttgcc

SEQ ID NO: 346 - DNA, 27 bp, synthetic construct
  misc_feature 1..27: note = K13X forward primer 2
  misc_feature 7: note = v is a, c, or g
  misc_feature 8: note = h is a, c, or t
  source 1..27: mol_type = other DNA
accattvhggtgaatctgatctttgcc

SEQ ID NO: 347 - DNA, 27 bp, synthetic construct
  misc_feature 1..27: note = K13X forward primer 3
  source 1..27: mol_type = other DNA
accatttgggtgaatctgatctttgcc

SEQ ID NO: 348 - DNA, 27 bp, synthetic construct
  misc_feature 1..27: note = K13X reverse primer 1
  misc_feature 8: note = h is a, c, or t
  misc_feature 9: note = n is a, c, g, or t
  source 1..27: mol_type = other DNA
attcacahnaatggtaacttcttcacg

SEQ ID NO: 349 - DNA, 27 bp, synthetic construct
  misc_feature 1..27: note = K13X reverse primer 2
  misc_feature 8: note = d is a, g, or t
  misc_feature 9: note = b is c, g, or t
  source 1..27: mol_type = other DNA
attcaccdbaatggtaacttcttcacg

SEQ ID NO: 350 - DNA, 27 bp, synthetic construct
  misc_feature 1..27: note = K13X reverse primer 3
  source 1..27: mol_type = other DNA
attcacccaaatggtaacttcttcacg

SEQ ID NO: 351 - DNA, 27 bp, synthetic construct
  misc_feature 1..27: note = K22X forward primer 1
  misc_feature 7: note = n is a, c, g, or t
  misc_feature 8: note = d is a, g, or t
  source 1..27: mol_type = other DNA
gacggcndtacccagaccgctgaattc

SEQ ID NO: 352 - DNA, 27 bp, synthetic construct
  misc_feature 1..27: note = K22X forward primer 2
  misc_feature 7: note = v is a, c, or g
  misc_feature 8: note = h is a, c, or t
  source 1..27: mol_type = other DNA
gacggcvhgacccagaccgctgaattc

SEQ ID NO: 353 - DNA, 27 bp, synthetic construct
  misc_feature 1..27: note = K22X forward primer 3
  source 1..27: mol_type = other DNA
gacggctggacccagaccgctgaattc

SEQ ID NO: 354 - DNA, 27 bp, synthetic construct
  misc_feature 1..27: note = K22X reverse primer 1
  misc_feature 8: note = h is a, c, or t
  misc_feature 9: note = n is a, c, g, or t
  source 1..27: mol_type = other DNA
ctgggtahngccgtcggcaaagatcag

SEQ ID NO: 355 - DNA, 27 bp, synthetic construct
  misc_feature 1..27: note = K22X reverse primer 2
  misc_feature 8: note = d is a, g, or t
  misc_feature 9: note = b is c, g, or t
  source 1..27: mol_type = other DNA
ctgggtcdbgccgtcggcaaagatcag

SEQ ID NO: 356 - DNA, 27 bp, synthetic construct
  misc_feature 1..27: note = K22X reverse primer 3
  source 1..27: mol_type = other DNA
ctgggtccagccgtcggcaaagatcag

SEQ ID NO: 357 - protein, 70 aa, synthetic construct
  REGION 1..70: note = FpL_C4KR_K7Q
ETPEEPQEEVTIRVNLIFADGRTQTAEFRGTFEEATAEAYRYADLLARVNGEYTADLEDGGYTINIRFAG

SEQ ID NO: 358 - protein, 70 aa, synthetic construct
  REGION 1..70: note = FpL_C4KR_K13V
ETPEEPREEVTIVVNLIFADGRTQTAEFRGTFEEATAEAYRYADLLARVNGEYTADLEDGGYTINIRFAG

SEQ ID NO: 359 - protein, 70 aa, synthetic construct
  REGION 1..70: note = FpL_C4K_K22T
ETPEEPREEVTIRVNLIFADGTTQTAEFRGTFEEATAEAYRYADLLARVNGEYTADLEDGGYTINIRFAG

SEQ ID NO: 360 - protein, 70 aa, synthetic construct; identical to SEQ ID NO: 137
  REGION 1..70: note = FpL_C4KR_K29P

SEQ ID NO: 361 - protein, 70 aa, synthetic construct
  REGION 1..70: note = FpL_C4KR_K29V
ETPEEPREEVTIRVNLIFADGRTQTAEFVGTFEEATAEAYRYADLLARVNGEYTADLEDGGYTINIRFAG

SEQ ID NO: 362 - protein, 70 aa, synthetic construct
  REGION 1..70: note = FpL_C4KR_K29I
ETPEEPREEVTIRVNLIFADGRTQTAEFIGTFEEATAEAYRYADLLARVNGEYTADLEDGGYTINIRFAG

SEQ ID NO: 363 - DNA, 30 bp, synthetic construct
  misc_feature 1..30: note = FpL_C3KX 7d_P6A forward primer
  source 1..30: mol_type = other DNA
ccaggagaggcggcggaagaagttaccatt

SEQ ID NO: 364 - DNA, 30 bp, synthetic construct
  misc_feature 1..30: note = FpL_C3KX 7d_P6A reverse primer
  source 1..30: mol_type = other DNA
ttcttccgccgcctctcctggtgtttccat

SEQ ID NO: 365 - protein, 70 aa, synthetic construct
  REGION 1..70: note = FpL_C3KX 7d_P6A
ETPGEAAEEVTIRVNLIFADGRIQTAEFIGTFEEATAEAYAYANLLARDYGDFTADLEDGGYTINIRFAG

SEQ ID NO: 366 - DNA, 30 bp, synthetic construct
  misc_feature 1..30: note = FpL_C3KX 7d_E8G forward primer
  source 1..30: mol_type = other DNA
gagtcagcgggcgaagttaccattcgcgtg

SEQ ID NO: 367 - DNA, 30 bp, synthetic construct
  misc_feature 1..30: note = FpL_C3KX 7d_E8G reverse primer
  source 1..30: mol_type = other DNA
ggtaacttcgcccgctgactctcctggtgt

SEQ ID NO: 368 - protein, 70 aa, synthetic construct
  REGION 1..70: note = FpL_C3KX 7d_E8G
ETPGESAGEVTIRVNLIFADGRIQTAEFIGTFEEATAEAYAYANLLARDYGDFTADLEDGGYTINIRFAG

SEQ ID NO: 369 - DNA, 30 bp, synthetic construct
  misc_feature 1..30: note = FpL_C3KX 7d_E8R forward primer
  source 1..30: mol_type = other DNA
gagtcagcgcgtgaagttaccattcgcgtg

SEQ ID NO: 370 - DNA, 30 bp, synthetic construct
  misc_feature 1..30: note = FpL_C3KX 7d_E8R reverse primer
  source 1..30: mol_type = other DNA
ggtaacttcacgcgctgactctcctggtgt

SEQ ID NO: 371 - protein, 70 aa, synthetic construct
  REGION 1..70: note = FpL_C3KX 7d_E8R
ETPGESAREVTIRVNLIFADGRIQTAEFIGTFEEATAEAYAYANLLARDYGDFTADLEDGGYTINIRFAG

SEQ ID NO: 372 - DNA, 27 bp, synthetic construct
  misc_feature 1..27: note = FpL_C3KX 7d_G21R forward primer
  source 1..27: mol_type = other DNA
gccgaccgtcggattcagaccgctgaa

SEQ ID NO: 373 - DNA, 27 bp, synthetic construct
  misc_feature 1..27: note = FpL_C3KX 7d_G21R reverse primer
  source 1..27: mol_type = other DNA
aatccgacggtcggcaaagatcagatt

SEQ ID NO: 374 - protein, 70 aa, synthetic construct
  REGION 1..70: note = FpL_C3KX 7d_G21R
ETPGESAEEVTIRVNLIFADRRIQTAEFIGTFEEATAEAYAYANLLARDYGDFTADLEDGGYTINIRFAG

SEQ ID NO: 375 - DNA, 30 bp, synthetic construct
  misc_feature 1..30: note = FpL_C3KX 7d_I23F forward primer
  source 1..30: mol_type = other DNA
gacggtcggtttcagaccgctgaattcatt

SEQ ID NO: 376 - DNA, 30 bp, synthetic construct
  misc_feature 1..30: note = FpL_C3KX 7d_I23F reverse primer
  source 1..30: mol_type = other DNA
agcggtctgaaaccgaccgtcggcaaagat

SEQ ID NO: 377 - protein, 70 aa, synthetic construct
  REGION 1..70: note = FpL_C3KX 7d_I23F
ETPGESAEEVTIRVNLIFADGRFQTAEFIGTFEEATAEAYAYANLLARDYGDFTADLEDGGYTINIRFAG

SEQ ID NO: 378 - DNA, 30 bp, synthetic construct
  misc_feature 1..30: note = FpL_C3KX 7d_I23L forward primer
  source 1..30: mol_type = other DNA
gacggtcggctgcagaccgctgaattcatt

SEQ ID NO: 379 - DNA, 30 bp, synthetic construct
  misc_feature 1..30: note = FpL_C3KX 7d_I23L reverse primer
  source 1..30: mol_type = other DNA
agcggtctgcagccgaccgtcggcaaagat

SEQ ID NO: 380 - protein, 70 aa, synthetic construct
  REGION 1..70: note = FpL_C3KX 7d_I23L
ETPGESAEEVTIRVNLIFADGRLQTAEFIGTFEEATAEAYAYANLLARDYGDFTADLEDGGYTINIRFAG

SEQ ID NO: 381 - DNA, 30 bp, synthetic construct
  misc_feature 1..30: note = FpL_C3KX 7d_E33V forward primer
  source 1..30: mol_type = other DNA
cgtacattcgtggaagccacagctgaagcc

SEQ ID NO: 382 - DNA, 30 bp, synthetic construct
  misc_feature 1..30: note = FpL_C3KX 7d_E33V reverse primer
  source 1..30: mol_type = other DNA
tgtggcttccacgaatgtaccaatgaattc

SEQ ID NO: 383 - protein, 70 aa, synthetic construct
  REGION 1..70: note = FpL_C3KX 7d_E33V
ETPGESAEEVTIRVNLIFADGRIQTAEFIGTFVEATAEAYAYANLLARDYGDFTADLEDGGYTINIRFAG

SEQ ID NO: 384 - DNA, 30 bp, synthetic construct
  misc_feature 1..30: note = FpL_C3KX 7d_K38H forward primer
  source 1..30: mol_type = other DNA
gccacagctcatgcctatgcttatgcgaat

SEQ ID NO: 385 - DNA, 30 bp, synthetic construct
  misc_feature 1..30: note = FpL_C3KX 7d_K38H reverse primer
  source 1..30: mol_type = other DNA
agcataggcatgagctgtggcttcttcgaa

SEQ ID NO: 386 - protein, 70 aa, synthetic construct
  REGION 1..70: note = FpL_C3KX 7d_K38H
ETPGESAEEVTIRVNLIFADGRIQTAEFIGTFEEATAHAYAYANLLARDYGDFTADLEDGGYTINIRFAG

SEQ ID NO: 387 - DNA, 30 bp, synthetic construct
  misc_feature 1..30: note = FpL_C3KX 7d_K38L forward primer
  source 1..30: mol_type = other DNA
gccacagctctggcctatgcttatgcgaat

SEQ ID NO: 388 - DNA, 30 bp, synthetic construct
  misc_feature 1..30: note = FpL_C3KX 7d_K38L reverse primer
  source 1..30: mol_type = other DNA
agcataggccagagctgtggcttcttcgaa

SEQ ID NO: 389 - protein, 70 aa, synthetic construct
  REGION 1..70: note = FpL_C3KX 7d_K38L
ETPGESAEEVTIRVNLIFADGRIQTAEFIGTFEEATALAYAYANLLARDYGDFTADLEDGGYTINIRFAG

SEQ ID NO: 390 - DNA, 30 bp, synthetic construct
  misc_feature 1..30: note = FpL_C3KX 7d_N44H forward primer
  source 1..30: mol_type = other DNA
gcttatgcgcatttgctggcccgtgattat

SEQ ID NO: 391 - DNA, 30 bp, synthetic construct
  misc_feature 1..30: note = FpL_C3KX 7d_N44H reverse primer
  source 1..30: mol_type = other DNA
ggccagcaaatgcgcataagcataggcttc

SEQ ID NO: 392 - protein, 70 aa, synthetic construct
  REGION 1..70: note = FpL_C3KX 7d_N44H
ETPGESAEEVTIRVNLIFADGRIQTAEFIGTFEEATAEAYAYAHLLARDYGDFTADLEDGGYTINIRFAG

SEQ ID NO: 393 - DNA, 30 bp, synthetic construct
  misc_feature 1..30: note = FpL_C3KX 7d_N44R forward primer
  source 1..30: mol_type = other DNA
gcttatgcgcgtttgctggcccgtgattat

SEQ ID NO: 394 - DNA, 30 bp, synthetic construct
  misc_feature 1..30: note = FpL_C3KX 7d_N44R reverse primer
  source 1..30: mol_type = other DNA
ggccagcaaacgcgcataagcataggcttc

SEQ ID NO: 395 - protein, 70 aa, synthetic construct
  REGION 1..70: note = FpL_C3KX 7d_N44R
ETPGESAEEVTIRVNLIFADGRIQTAEFIGTFEEATAEAYAYARLLARDYGDFTADLEDGGYTINIRFAG

SEQ ID NO: 396 - DNA, 30 bp, synthetic construct
  misc_feature 1..30: note = FpL_C3KX 7d_R48H forward primer
  source 1..30: mol_type = other DNA
ttgctggcccatgattatggtgactttacg

SEQ ID NO: 397 - DNA, 30 bp, synthetic construct
  misc_feature 1..30: note = FpL_C3KX 7d_R48H reverse primer
  source 1..30: mol_type = other DNA
aacataatcatgggccagcaaattcgcata

SEQ ID NO: 398 - protein, 70 aa, synthetic construct
  REGION 1..70: note = FpL_C3KX 7d_R48H
ETPGESAEEVTIRVNLIFADGRIQTAEFIGTFEEATAEAYAYANLLAHDYGDFTADLEDGGYTINIRFAG

SEQ ID NO: 399 - DNA, 30 bp, synthetic construct
  misc_feature 1..30: note = FpL_C3KX 7d_N50M forward primer
  source 1..30: mol_type = other DNA
gcccgtgatatgggtgactttacggcggac

SEQ ID NO: 400 - DNA, 30 bp, synthetic construct
  misc_feature 1..30: note = FpL_C3KX 7d_N50M reverse primer
  source 1..30: mol_type = other DNA
aaagtcacccatatcacgggccagcaaatt

SEQ ID NO: 401 - protein, 70 aa, synthetic construct
  REGION 1..70: note = FpL_C3KX 7d_N50M
ETPGESAEEVTIRVNLIFADGRIQTAEFIGTFEEATAEAYAYANLLARDMGDFTADLEDGGYTINIRFAG

SEQ ID NO: 402 - DNA, 30 bp, synthetic construct
  misc_feature 1..30: note = FpL_C3KX 7d_E52Y forward primer
  source 1..30: mol_type = other DNA
gattatggttattttacggcggacctggaa

SEQ ID NO: 403 - DNA, 30 bp, synthetic construct
  misc_feature 1..30: note = FpL_C3KX 7d_E52Y reverse primer
  source 1..30: mol_type = other DNA
cgccgtaaaataaccataatcacgggccag

SEQ ID NO: 404 - protein, 70 aa, synthetic construct
  REGION 1..70: note = FpL_C3KX 7d_E52Y
ETPGESAEEVTIRVNLIFADGRIQTAEFIGTFEEATAEAYAYANLLARDYGYFTADLEDGGYTINIRFAG

SEQ ID NO: 405 - DNA, 30 bp, synthetic construct
  misc_feature 1..30: note = FpL_C3KX 7d_Y53S forward primer
  source 1..30: mol_type = other DNA
tatggtgactctacggcggacctggaagat

SEQ ID NO: 406 - DNA, 30 bp, synthetic construct
  misc_feature 1..30: note = FpL_C3KX 7d_Y53S reverse primer
  source 1..30: mol_type = other DNA
gtccgccgtagagtcaccataatcacgggc

SEQ ID NO: 407 - protein, 70 aa, synthetic construct
  REGION 1..70: note = FpL_C3KX 7d_Y53S
ETPGESAEEVTIRVNLIFADGRIQTAEFIGTFEEATAEAYAYANLLARDYGDSTADLEDGGYTINIRFAG

SEQ ID NO: 408 - protein, 70 aa, synthetic construct
  REGION 1..70: note = FpL_C3KX 9a
ETPGESAEEVTIRVNLIFADGRRQTAEFIGTFEEATAEAYAYARLLARDYGEFTADLEDGGYTINIRFVG

SEQ ID NO: 409 - protein, 70 aa, synthetic construct
  REGION 1..70: note = FpL_C3KX 9b
ETPGESAEEVTIRVNLIFADGRRQTAEFIGTFEEATAEAYAYAHLLARDYGEFTADLEDGGYTINIRFVG

SEQ ID NO: 410 - protein, 70 aa, synthetic construct
  REGION 1..70: note = FpL_C3KX 9c
ETPGESAEEVTIRVNLIFADGRRQTAEFIGTFEEATAEAYAYANLLARDYGEFTADLEDGGYTLNIRFVG

SEQ ID NO: 411 - protein, 70 aa, synthetic construct
  REGION 1..70: note = FpL_C3KX 9d
ETPGESAEEVTIRVNLIFADGRIQTAEFIGTFEEATAEAYAYARLLARDYGEFTADLEDGGYTLNIRFVG

SEQ ID NO: 412 - protein, 70 aa, synthetic construct
  REGION 1..70: note = FpL_C3KX 9e
ETPGESAEEVTIRVNLIFADGRIQTAEFIGTFEEATAEAYAYAHLLARDYGEFTADLEDGGYTLNIRFVG

SEQ ID NO: 413 - protein, 70 aa, synthetic construct
  REGION 1..70: note = FpL_C3KX 10a
ETPGESAEEVTIRVNLIFADGRRQTAEFIGTFEEATAEAYAYARLLAHDYGEFTADLEDGGYTLNIRFVG

SEQ ID NO: 414 - protein, 70 aa, synthetic construct
  REGION 1..70: note = FpL_C3KX 10b
ETPGESAEEVTIRVNLIFADGRRQTAEFIGTFEEATAEAYAYAHLLAHDYGEFTADLEDGGYTLNIRFVG

SEQ ID NO: 415 - DNA, 210 bp, synthetic construct
  misc_feature 1..210: note = FpL_C3KX 9a_DNA
  source 1..210: mol_type = other DNA
gaaacaccgggagagagcgccgaagaggtgaccattcgtgtaaatttgattttcgccgacggtcgccgccagacggctgagttcattggtaccttcgaggaagcgacggcagaggcttatgcgtacgcgcgtttactggcccgcgattacggtgagtttacagcagatctggaggatggcggctacaccatcaacattcgctttgtgggt

SEQ ID NO: 416 - DNA, 210 bp, synthetic construct
  misc_feature 1..210: note = FpL_C3KX 9b_DNA
  source 1..210: mol_type = other DNA
gaaacaccgggagagagcgccgaagaggtgaccattcgtgtaaatttgattttcgccgacggtcgccgccagacggctgagttcattggtaccttcgaggaagcgacggcagaggcttatgcgtacgcgcatttactggcccgcgattacggtgagtttacagcagatctggaggatggcggctacaccatcaacattcgctttgtgggt

SEQ ID NO: 417 - DNA, 210 bp, synthetic construct
  misc_feature 1..210: note = FpL_C3KX 9c_DNA
  source 1..210: mol_type = other DNA
gaaacaccgggagagagcgccgaagaggtgaccattcgtgtaaatttgattttcgccgacggtcgccgccagacggctgagttcattggtaccttcgaggaagcgacggcagaggcttatgcgtacgcgaacttactggcccgcgattacggtgagtttacagcagatctggaggatggcggctacaccttaaacattcgctttgtgggt

SEQ ID NO: 418 - DNA, 210 bp, synthetic construct
  misc_feature 1..210: note = FpL_C3KX 9d_DNA
  source 1..210: mol_type = other DNA
gaaacaccgggagagagcgccgaagaggtgaccattcgtgtaaatttgattttcgccgacggtcgcattcagacggctgagttcattggtaccttcgaggaagcgacggcagaggcttatgcgtacgcgcgcttactggcccgcgattacggtgagtttacagcagatctggaggatggcggctacaccttaaacattcgctttgtgggt

SEQ ID NO: 419 - DNA, 210 bp, synthetic construct
  misc_feature 1..210: note = FpL_C3KX 9e_DNA
  source 1..210: mol_type = other DNA
gaaacaccgggagagagcgccgaagaggtgaccattcgtgtaaatttgattttcgccgacggtcgcattcagacggctgagttcattggtaccttcgaggaagcgacggcagaggcttatgcgtacgcgcatttactggcccgcgattacggtgagtttacagcagatctggaggatggcggctacaccttaaacattcgctttgtgggt

SEQ ID NO: 420 - DNA, 210 bp, synthetic construct
  misc_feature 1..210: note = FpL_C3KX 10a_DNA
  source 1..210: mol_type = other DNA
gaaacaccgggagagagcgccgaagaggtgaccattcgtgtaaatttgattttcgccgacggtcgccgccagacggctgagttcattggtaccttcgaggaagcgacggcagaggcttatgcgtacgcgcgcttactggcccatgattacggtgagtttacagcagatctggaggatggcggctacaccttaaacattcgctttgtgggt

SEQ ID NO: 421 - DNA, 210 bp, synthetic construct
  misc_feature 1..210: note = FpL_C3KX 10b_DNA
  source 1..210: mol_type = other DNA
gaaacaccgggagagagcgccgaagaggtgaccattcgtgtaaatttgattttcgccgacggtcgccgccagacggctgagttcattggtaccttcgaggaagcgacggcagaggcttatgcgtacgcgcatttactggcccatgattacggtgagtttacagcagatctggaggatggcggctacaccttaaacattcgctttgtgggt

SEQ ID NO: 422 - DNA, 30 bp, synthetic construct
  misc_feature 1..30: note = N15X forward primer 1
  misc_feature 10: note = n is a, c, g, or t
  source 1..30: mol_type = other DNA
attcgtgtgndtttaatcttcgctgatggt

SEQ ID NO: 423 - DNA, 30 bp, synthetic construct
  misc_feature 1..30: note = N15X forward primer 2
  source 1..30: mol_type = other DNA
attcgtgtgvhgttaatcttcgctgatggt

SEQ ID NO: 424 - DNA, 30 bp, synthetic construct
  misc_feature 1..30: note = N15X forward primer 3
  source 1..30: mol_type = other DNA
attcgtgtgtggttaatcttcgctgatggt

SEQ ID NO: 425 - DNA, 30 bp, synthetic construct
  misc_feature 1..30: note = N15X reverse primer 1
  misc_feature 12: note = n is a, c, g, or t
  source 1..30: mol_type = other DNA
cacacgaatahncacacgaatggtgacctc

SEQ ID NO: 426 - DNA, 30 bp, synthetic construct
  misc_feature 1..30: note = N15X reverse primer 2
  source 1..30: mol_type = other DNA
cacacgaatcdbcacacgaatggtgacctc

SEQ ID NO: 427 - DNA, 30 bp, synthetic construct
  misc_feature 1..30: note = N15X reverse primer 3
  source 1..30: mol_type = other DNA
cacacgaatccacacacgaatggtgacctc

SEQ ID NO: 428 - DNA, 30 bp, synthetic construct
  misc_feature 1..30: note = E34X forward primer 1
  misc_feature 10: note = n is a, c, g, or t
  source 1..30: mol_type = other DNA
acgtttgaandtgcaaccgccgaagcgtac

SEQ ID NO: 429 - DNA, 30 bp, synthetic construct
  misc_feature 1..30: note = E34X forward primer 2
  source 1..30: mol_type = other DNA
acgtttgaavhggcaaccgccgaagcgtac

SEQ ID NO: 430 - DNA, 30 bp, synthetic construct
  misc_feature 1..30: note = E34X forward primer 3
  source 1..30: mol_type = other DNA
acgtttgaatgggcaaccgccgaagcgtac

SEQ ID NO: 431 - DNA, 30 bp, synthetic construct
  misc_feature 1..30: note = E34X reverse primer 1
  misc_feature 12: note = n is a, c, g, or t
  source 1..30: mol_type = other DNA
ttcaaacgtahnttcaaacgtcccaatgaa

SEQ ID NO: 432 - DNA, 30 bp, synthetic construct
  misc_feature 1..30: note = E34X reverse primer 2
  source 1..30: mol_type = other DNA
ttcaaacgtcdbttcaaacgtcccaatgaa

SEQ ID NO: 433 - DNA, 30 bp, synthetic construct
  misc_feature 1..30: note = E34X reverse primer 3
  source 1..30: mol_type = other DNA
ttcaaacgtccattcaaacgtcccaatgaa

SEQ ID NO: 434 - protein, 70 aa, synthetic construct
  REGION 1..70: note = FpL_C3KX 7e_N15V
ETPGESAEEVTIRVVLIFADGRIQTAEFIGTFEEATAEAYAYANLLARDYGEFTADLEDGGYTINIRFVG

SEQ ID NO: 435 - protein, 70 aa, synthetic construct
  REGION 1..70: note = FpL_C3KX 7e_E34D
ETPGESAEEVTIRVNLIFADGRIQTAEFIGTFEDATAEAYAYANLLARDYGEFTADLEDGGYTINIRFVG

SEQ ID NO: 436 - protein, 70 aa, synthetic construct
  REGION 1..70: note = FpL_C3KX 7e_E34F
ETPGESAEEVTIRVNLIFADGRIQTAEFIGTFEFATAEAYAYANLLARDYGEFTADLEDGGYTINIRFVG

SEQ ID NO: 437 - protein, 70 aa, synthetic construct
  REGION 1..70: note = FpL_C3KX 7e_E34L
ETPGESAEEVTIRVNLIFADGRIQTAEFIGTFELATAEAYAYANLLARDYGEFTADLEDGGYTINIRFVG

SEQ ID NO: 438 - protein, 70 aa, synthetic construct
  REGION 1..70: note = FpL_C3KX 7e_E34V
ETPGESAEEVTIRVNLIFADGRIQTAEFIGTFEVATAEAYAYANLLARDYGEFTADLEDGGYTINIRFVG